European Patent Application EP 4 167 249 A1, published April 19, 2023. Title: APPARATUS, METHOD AND RECORDING MEDIUM STORING COMMAND FOR DETERMINING GUT MICROBIOME INDEX. Applicant: CHUNLAB, INC. The sequence listing filed with the application follows.

SEQUENCE LISTING (76 sequences)

SEQ ID NO: 1 - DNA, 1486 bp, Unknown
  16S rRNA(Bacteroides genus)
agagtttgatcctggctcaggatgaacgctagctacaggcttaacacatgcaagtcgaggggcagcatggtcttagcttgctaaggccgatggcgaccggcgcacgggtgagtaacacgtatccaacctgccgtctactcttggacagccttctgaaaggaagattaatacaagatggcatcatgagtccgcatgttcacatgattaaaggtattccggtagacgatggggatgcgttccattagatagtaggcggggtaacggcccacctagtcttcgatggataggggttctgagaggaaggtcccccacattggaactgagacacggtccaaactcctacgggaggcagcagtgaggaatattggtcaatgggcgagagcctgaaccagccaagtagcgtgaaggatgactgccctatgggttgtaaacttcttttataaaggaataaagtcgggtatgcatacccgtttgcatgtactttatgaataaggatcggctaactccgtgccagcagccgcggtaatacggaggatccgagcgttatccggatttattgggtttaaagggagcgtagatggatgtttaagtcagttgtgaaagtttgcggctcaaccgtaaaattgcagttgatactggatatcttgagtgcagttgaggcaggcggaattcgtggtgtagcggtgaaatgcttagatatcacgaggaactccgattgcgaaggcagcctgctaagctgcaactgacattgaggctcgaaagtgtgggtatcaaacaggattagataccctggtagtccacacggtaaacgatgaatactcgctgtttgcgatatacggcaagcggccaagcgaaagcgttaagtattccacctggggagtacgccggcaacggtgaaactcaaaggaattgacgggggcccgcacaagcggaggaacatgtggtttaattcgatgatacgcgaggaaccttacccgggcttaaattgcagatgaattacggtgaaagccgtaagccgcaaggcatctgtgaaggtgctgcatggttgtcgtcagctcgtgccgtgaggtgtcggcttaagtgccataacgagcgcaacccttgttgtcagttactaacaggttctgctgaggactctgacaagactgccatcgtaagatgtgaggaaggtggggatgacgtcaaatcagcacggcccttacgtccggggctacacacgtgttacaatggggggtacagagggccgctaccacgcgagtggatgccaatcccaaaaacctctctcagttcggactggagtctgcaacccgactccacgaagctggattcgctagtaatcgcgcatcagccacggcgcggtgaatacgttcccgggccttgtacacaccgcccgtcaagccatgggagccgggggtacctgaagtgcgtaaccgcgaggagcgccctagggtaaaactggtgactggggctaagtcgtaacaaggta

SEQ ID NO: 2 - DNA, 1486 bp, Unknown; identical to SEQ ID NO: 1
  16S rRNA(Bilophila genus)

SEQ ID NO: 3 - DNA, 1481 bp, Unknown
  16S rRNA(Butyricicoccus genus)
agtttgatcctggctcaggatgaacgctggcggcgtgcctaacacatgcaagtcgaacggagttgtttgaggaaatccttcgggatggaatcttccaacttagtggcggacgggtgagtaacgcgtgagcaatctgcctttcagagggggataacagccggaaacggctgctaataccgcataatgcattgaattcgcatgtttttgatgccaaagattttatcgctgaaagatgagctcgcgtctgattagctagttggcggggtaacggcccaccaaggcgacgatcagtagccggactgagaggttgaacggccacattgggactgaggacacggcccagactcctaccgggaggcagcagtggggaatattgcgcaatgggggcaaccctgacgcagcaacgccgcgtgattgatgaaggtcttcggattgtaaaaatctttaatcagggacgaaacaaatgacggtacctgaagaataagctccggctaactacgtgccagcagccgcggtaatacgtagggagcaagcgttatccggatttactgggtgtaaagggcgtgtaggcgggcttgtaagttggaagtgaaatctcggggcttaaccccgaaactgctttcaaaactgcgagtcttgagtgatggagaggcaggcggaattcccagtgtagcggtgaaatgcgtagatattgggaggaacaccagtggcgaaggcggcctgctggacattaactgacgctgaggcgcgaaagcgtggggagcaaacaggattagataccctggtagtccacgccgtaaacgatggatactaggtgtgggaggtattgaccccttccgtgccggagttaacacaataagtatcccacctggggagtacggccgcaaggttgaaactcaaaggaattgacgggggcccgcacaagcagtggagtatgtggtttaattcgaagcaacgcgcaagaaccttaccaagtcttgacatcccgatgaccgctcyagagatagggcttttcttcggaacatcggtgacaggtggtgcatggttgtcgtcagctcgtgtcgtgagatgttgggttaagtcccgcaacgagcgcaacccttacgggttagttgctacgcaagagcactctagccggactgccgttgacaaaacggaggaaggtggggacgacgtcaaatcatcatgccccttatgacttgggctacacacgtactacaatggcagtcatacagagggaagcaaaaccgcgaggtggagcaaatccctaaaagctgtcccagttcagattgcaggctgcaactcgcctgcatgaagtcggaattgctagtaatcgcggatcagcatgccgcggtgaatacgttcccgggccttgtacacaccgcccgtcacaccatgagagccggtaatacccgaagtccgtagtctaaccgcaaggaggacgcggccgaaggtaggactggtaattgggacgaagtcgt

SEQ ID NO: 4 - DNA, 1483 bp, Unknown
  16S rRNA(Butyricimonas genus)
agagtttgatcctggctcaggatgaacgctagcgacaggcttaacacatgcaagtcgaggggcagcggggagtagcaatacttggccggcgaccggcgcacgggtgagtaacacgtgtgcaaccaaccccgtaccgggagataacccgcggaaacgtggactaacatcccataacactgtataatcgcatggttatgcatttaaaattccggtggtacgggacgggcacgcgcgacattaggtagttggcggggtaacggcccaccaagccgacgatgtctaggggttctgagaggaaggtcccccacactggaactgagacacggtccagactcctacgggaggcagcagtgaggaatattggtcaatgggcgagagcctgaaccagccaagtcgcgtgagggaagaatggtctatggcctgtaaacctcttttgccagggaagaataaatggcacgcgtgccatcttgccagtacctgacgaataagcatcggctaactccgtgccagcagccgcggtaatacgggggatgcgagcgttatccggatttattgggtttaaagggcgcgtaggcgggacgccaagtcagcggtaaaagactgcagctaaactgtagcacgccgttgaaactggcgacctggagacgagacgagggaggcggaacaagtgaagtagcggtgaaatgcttagatatcacttggaaccccgatagcgaaggcagcttcccaggctcgatctgacgctgatgcgcgagagcgtgggtagcgaacaggattagataccctggtagtccacgccgtaaacgatgctcactggatcttggcgatacaccgccagggttcaagcgaaagtattaagtgagccacctggggagtacgtcggcaacgatgaaactcaaaggaattgacgggggcccgcacaagcggaggaacatgtggtttaattcgatgatacgcgaggaaccttacccgggtttaaatgtggagtgcatgagctggaaacagttctttccctcgggactcttcacaaggtgctgcatggttgtcgtcagctcgtgccgtgaggtgtcgggttaagtcccataacgagcgcaacccctatcgccagttgccagcggttgaggccgggcactctgtcgagactgccaccgtaaggtgcgaggaaggcggggatgacgtcaaatcagcacggcccttacacccggggcgacacacgtgttacaatggccggtacagagggcagccacggggtgacccggagcgaatctctaaagccggtcgtagttcggactggagtctgcaacccgactccacgaagttggattcgctagtaatcgcgcatcagccatggcgcggtgaatacgttcccgggccttgtacacaccgcccgtcaagccatggaagccgggagtacctgaagatcgtgaccgcgaggaacgggctagggtaataccggtaactggggctaagtcgtaacaaggta

SEQ ID NO: 5 - DNA, 1450 bp, Unknown
  16S rRNA(Clostridium_g24)
gatgaacgctggcggcgtgcttaacacatgcaagtcgagcgaagcaatttaaatgagacttcggtggattttaaattgactgagcggcggacgggtgagtaacgcgtggataacctgcctcacacagggggataacagttagaaatgactgctaataccgcataagcgcacggtaccgcatggtacagtgcgaaaaactccggtggtgtgagatggatccgcgtctgattaggtagttggtgaggtaacggcccaccaagccgacgatcagtagccgacctgagagggtgaccggccacattgggactgagacacggcccaaactcctacgggaggcagcagtggggaatattgcacaatgggcgaaagcctgatgcagcaacgccgcgtgagtgaagaagtatctcggtatgtaaagctctatcagcagggaagaaaatgacggtacctgactaagaagccccggctaactacgtgccagcagccgcggtaatacgtagggggcaagcgttatccggatttactgggtgtaaagggagcgcagacggcactgcaagtctgaagtgaaagcccggggctcaaccccgggactgctttggaaactgtagagctagagtgctggagaggcaagcggaattcctagtgtagcggtgaaatgcgtagatattaggaagaacaccagtggcgaaggcggcttgctggacagtaactgacgttcaggctcgaaagcgtggggagcaaacaggattagataccctggtagtccacgccgtaaacgatgaatactaggtgttggtgggcaaagcccatcggtgccgccgcaaacgcaataagtattccacctggggagtacgttcgcaagaatgaaactcaaaggaattgacggggacccgcacaagcggtggagcatgtggtttaattcgaagcaacgcgaagaaccttaccaagtcttgacatcgtgatgaccggaacttaaccgttccttcccttcggggcatcatagacaggtggtgcatggttgtcgtcagctcgtgtcgtgagatgttgggttaagtcccgcaacgagcgcaacccttatcctcagtagccagcagtaagatgggcactctggggagactgccagggataacctggaggaaggtggggatgacgtcaaatcatcatgccccttatgatttgggctacacacgtgctacaatggcgtaaacaaagggaagcaagagggcgacctggagcaaatcccaaaaataacgtcccagttcggactgtagtctgcaacccgactacacgaagctggaatcgctagtaatcgcagatcagaatgctgcggtgaatacgttcccgggtcttgtacacaccgcccgtcacaccatgggagtcagcaacgcccgaagtcagtgactcaaccgcaaggagagagctgccgaaggcggggcaggtaactggggtg

SEQ ID NO: 6 - DNA, 1471 bp, Unknown
  16S rRNA(Clostridium_g35)
agagtttgatcctggctcaggatgaacgctggcggcgtgcctaacacatgcaagtcgaacgaagcgatttaacggaagttttcggatggaagttgaattgactgagtggcggacgggtgagtaacgcgtgggtaacctgccttgtactgggggacaacagttagaaatgactgctaataccgcataagcgcacagtattgcatgatacagtgtgaaaaactccggtggtacaagatggacccgcgtctgattagctagttggtaaggtaacggcttaccaaggcgacgatcagtagccgacctgagagggtgaccggccacattgggactgagacacggccnnaactcctacgggaggcagcagtggggaatattgcacaatgggcgaaagcctgatgcagcgacgccgcgtgagtgaagaagtatttcggtatgtaaagctctatcagcagggaagaaaatgacggtacctgactaagaagccccggctaactacgtgccagcagccgcggtaatacgtagggggnnagcgttatccggatttactgggtgtaaagggagcgtagacggtaaagcaagtctgaagtgaaagcccgcgnctcaactgcggnnctgctttggaaactgtttaactggagtgtcggagaggtaagtggaattcctagtgtagcggtgaaatgcgtagatattaggaggaacacnagtggcgaaggcgacttactggacgataactgacgttgaggctcgaaagcgtggggagcaaacaggattagataccctggtagtccacgccgtaaacgatgaatactaggtgttggggagcaaagctcttcggtgccgtcgcaaacgcagtaagtattccacctggggagtacgttcgcaagaatgaaactcaaaggaattgacggggaccngcacaagcggtggagcatgtggtttaattcgaannaacgcgaagaaccttaccaggtcttgacatcgactcgacgggggagtaacgtcccnntnccttcggggcggagaagacaggtggtgcatggttgtcgtcagctcgtgtcgtgagatgttgggttnagtcccgcaacgagcgcaacccttattctaagtagccagcggttcggccgggaactcttgggagactgccagggataacctggaggaaggtggggatgacgtcnaatcatcatgccccttatgatctgggctacacacgtgctacaatggcgtaaacanagagaagcaagaccgcgaggtggagcaaatctcaaaaataacgtctcagttcggactgcaggctgcaactcgcctgcacgaagctggaatcgctagtaatcgcgaatcagaatgtcgcggtgaatacgttcccgggtcttgtacacaccgnncgtcacaccatgggagtcagtaacgcccgaagtcagtgacccaaccgcaaggagggagctgccgaaggcgggaccganaacnnggg

SEQ ID NO: 7 - DNA, 1485 bp, Unknown
  16S rRNA(Clostridium_g6)
agagtttgatcctggctcaggatgaacgctggcggcgtgcctaatacatgcaagtcgaacgcgagcacttgtgctcgagtggcgaacgggtgagtaatacataagtaacctgccctagacagggggataactattggaaacgatagctaagaccgcataggtacggacactgcatggtgaccgtattaaaagtgcctcaaagcactggtagaggatggacttatggcgcattagctggttggcggggtaacggcccaccaaggcgacgatgcgtagccgacctgagagggtgaccggccacactgggactgagacacggcccagactcctacgggaggcagcagtagggaattttcggcaatgggggaaaccctgaccgagcaacgccgcgtgaaggaagaaggttttcggattgtaaacttctgttataaaggaagaacggcggctacaggaaatggtagccgagtgacggtactttattagaaagccacggctaactacgtgccagcagccgcggtaatacgtaggtggcaagcgttatccggaattattgggcgtaaagagggagcaggcggcagcaagggtctgtggtgaaagcctgaagcttaacttcagtaagccatagaaaccaggcagctagagtgcaggagaggatcgtggaattccatgtgtagcggtgaaatgcgtagatatatggaggaacaccagtggcgaaggcgacgatctggcctgcaactgacgctcagtcccgaaagcgtggggagcaaataggattagataccctagtagtccacgccgtaaacgatgagtactaagtgttggatgtcaaagttcagtgctgcagttaacgcaataagtactccgcctgagtagtacgttcgcaagaatgaaactcaaaggaattgacgggggcccgcacaagcggtggagcatgtggtttaattcgaagcaacgcgaagaaccttaccaggtcttgacatactcataaaggctccagagatggagagatagctatatgagatacaggtggtgcatggttgtcgtcagctcgtgtcgtgagatgttgggttaagtcccgcaacgagcgcaacccttatcgttagttaccatcattaagttggggactctagcgagactgccagtgacaagctggaggaaggcggggatgacgtcaaatcatcatgccccttatgacctgggctacacacgtgctacaatggatggtgcagagggaagcgaagccgcgaggtgaagcaaaacccataaaaccattctcagttcggattgtagtctgcaactcgactacatgaagttggaatcgctagtaatcgcgaatcagcatgtcgcggtgaatacgttctcgggccttgtacacaccgcccgtcacaccacgagagttgataacacccgaagccggtggcctaaccgcaaggaaggagctgtctaaggtgggattgatgattggggtgaagtcgtaacaaggta

SEQ ID NO: 8 - DNA, 1553 bp, Unknown
  16S rRNA(Enterococcus genus)
agagtttgatcctggctcaggacgaacgctggcggcgtgcctaatacatgcaagtcgaacgcttctttttccaccggagcttgctccaccggaaaaagaggagtggcgaacgggtgagtaacacgtgggtaacctgcccatcagaaggggataacacttggaaacaggtgctaataccgtataacaatcgaaaccgcatggttttgatttgaaaggcgctttcgggtgtcgctgatggatggacccgcggtgcattagctagttggtgaggtaacggctcaccaaggccacgatgcatagccgacctgagagggtgatcggccacattgggactgagacacggcccaaactcctacgggaggcagcagtagggaatcttcggcaatggacgaaagtctgaccgagcaacgccgcgtgagtgaagaaggttttcggatcgtaaaactctgttgttagagaagaacaaggatgagagtaactgttcatcccttgacggtatctaaccagaaagccacggctaactacgtgccagcagccgcggtaatacgtaggtggcaagcgttgtccggatttattgggcgtaaagcgagcgcaggcggtttcttaagtctgatgtgaaagcccccggctcaaccggggagggtcattggaaactgggagacttgagtgcagaagaggagagtggaattccatgtgtagcggtgaaatgcgtagatatatggaggaacaccagtggcgaaggcggctctctggtctgtaactgacgctgaggctcgaaagcgtggggagcaaacaggattagataccctggtagtccacgccgtaaacgatgagtgctaagtgttggagggtttccgcccttcagtgctgcagctaacgcattaagcactccgcctggggagtacgaccgcaaggttgaaactcaaaggaattgacgggggcccgcacaagcggtggagcatgtggtttaattcgaagcaacgcgaagaaccttaccaggtcttgacatcctttgaccactctagagatagagcttccccttcgggggcaaagtgacaggtggtgcatggttgtcgtcagctcgtgtcgtgagatgttgggttaagtcccgcaacgagcgcaacccttattgttagttgccatcattcagttgggcactctagcaagactgccggtgacaaaccggaggaaggtggggatgacgtcaaatcatcatgccccttatgacctgggctacacacgtgctacaatgggaagtacaacgagttgcgaagtcgcgaggctaagctaatctcttaaagcttctctcagttcggattgcaggctgcaactcgcctgcatgaagccggaatcgctagtaatcgcggatcagcacgccgcggtgaatacgttcccgggccttgtacacaccgcccgtcacaccacgagagtttgtaacacccgaagtcggtgaggtaaccttttggagccagccgcctaaggtgggatagatgattggggtgaagtcgtaacaaggtagccgtatcggaaggtgcggctggatcacctccttt

SEQ ID NO: 9 - DNA, 1556 bp, Unknown
  16S rRNA(Lactobacillus genus)
agagtttgatcctggctcaggacgaacgctggcggcgtgcctaatacatgcaagtcgaacgaagctttctttcaccgaatgcttgcattcaccgaaagaagcttagtggcgaacgggtgagtaacacgtaggcaacctgcccaaaagagggggataacacttggaaacaggtgctaataccgcataaccatgaacaccgcatgatgttcatgtaaaagacggcttttgctgtcacttttggatgggcctgcggcgtattaacttgttggtggggtaatggcctaccaaggtgatgatacgtagccgaactgagaggttgatcggccacattgggactgagacacggcccaaactcctacgggaggcagcagtagggaatcttccacaatggacgaaagtctgatggagcaacgccgcgtgaatgaagaaggccttcgggtcgtaaaattctgttgtcagagaagaacgtgcgtgagagtaactgttcacgtattgacggtatctgaccagaaagccacggctaactacgtgccagcagccgcggtaatacgtaggtggcgagcgttgtccggatttattgggcgtaaagggaacgcaggcggtcttttaagtctgatgtgaaagccttcggcttaaccgaagtagtgcattggaaactggaagacttgagtgcagaagaggagagtggaactccatgtgtagcggtgaaatgcgtagatatatggaagaacaccagtggcgaaagcggctctctggtctgtaactgacgctgaggttcgaaagcgtgggtagcaaacaggattagataccctggtagtccacgccgtaaacgatgagtgctaagtgttggagggtttccgcccttcagtgctgcagctaacgcattaagcactccgcctggggagtacggtcgcaagactgaaactcaaaggaattgacgggggcccgcacaagcggtggagcatgtggtttaattcgaagcaacgcgaagaaccttaccaggtcttgacatcttctgacaattccagagatggaacgttcccttcggggacagaatgacaggtggtgcatggttgtcgtcagctcgtgtcgtgagatgttgggttaagtcccgcaacgagcgcaacccttattgtcagttgccatcattaagttgggcactctggcgagactgccggtgacaaaccggaggaaggtggggatgacgtcaaatcatcatgccccttatgacctgggctacacacgtgctacaatggacggtacaacgagtcgctaactcgcgagggcaagctaatctcttaaagccgttctcagttcggattgcaggctgcaactcgcctgcatgaagtcggaatcgctagtaatcgcgaatcagcatgtcgcggtgaatacgttcccgggccttgtacacaccgcccgtcacaccatgagagtttgtaacacccaaagtcggtggggtaaccttttggagccagccgcctaaggtgggacagatgattggggtgaagtcgtaacaaggtagccgtaggagaacctgcggctggatcacctccttt

SEQ ID NO: 10 - DNA, 1522 bp, Unknown
  16S rRNA(Megasphaera genus)
agagtttgatcctggctcaggacgaacgctggcggcgtgcttaacacatgcaagtcgaacgagaagagatgagaagcttgcttcttatcaattcgagtggcaaacgggtgagtaacgcgtaagcaacctgcccttcagatggggacaacagctggaaacggctgctaataccgaatacgttctttttgtcgcatggcagagggaagaaagggaggctcttcggagctttcgctgaaggaggggcttgcgtctgattagctagttggaggggtaacggcccaccaaggcgacgatcagtagccggtctgagaggatgaacggccacattgggactgagacacggcccagactcctacgggaggcagcagtggggaatcttccgcaatggacgaaagtctgacggagcaacgccgcgtgaacgatgacggccttcgggttgtaaagttctgttatacgggacgaatggcgtagcggtcaatacccgttacgagtgacggtaccgtaagagaaagccacggctaactacgtgccagcagccgcggtaatacgtaggtggcaagcgttgtccggaattattgggcgtaaagggcgcgcaggcggcgtcgtaagtcggtcttaaaagtgcggggcttaaccccgtgaggggaccgaaactgcgatgctagagtatcggagaggaaagcggaattcctagtgtagcggtgaaatgcgtagatattaggaggaacaccagtggcgaaagcggctttctggacgacaactgacgctgaggcgcgaaagccaggggagcaaacgggattagataccccggtagtcctggccgtaaacgatggatactaggtgtaggaggtatcgaccccttctgtgccggagttaacgcaataagtatcccgcctggggagtacggccgcaaggctgaaactcaaaggaattgacgggggcccgcacaagcggtggagtatgtggtttaattcgacgcaacgcgaagaaccttaccaagccttgacattgattgctatggatagagatatccagttcctcttcggaggacaagaaaacaggtggtgcacggctgtcgtcagctcgtgtcgtgagatgttgggttaagtcccgcaacgagcgcaacccctatcttctgttaccagcggttcggccggggactcaggagagactgccgcagacaatgcggaggaaggcggggatgacgtcaagtcatcatgccccttatggcttgggctacacacgtactacaatggctcttaatagagggaagcgaaggagcgatccggagcaaaccccaaaaacagagtcccagttcggattgcaggctgcaactcgcctgcatgaagcaggaatcgctagtaatcgcaggtcagcatactgcggtgaatacgttcccgggccttgtacacaccgcccgtcacaccacgaaagtcattcacacccgaagccggtgaggtaaccttttggagccagccgtcgaaggtgggggcgatgattggggtgaagtcgtaacaaggta

SEQ ID NO: 11 - DNA, 1491 bp, Unknown
  16S rRNA(PAC000740_g)
agagtttgatcctggctcaggatgaacgctggcggcgtgcttaacacatgcaagtcgagcgaagcactctgctttgaatctttcgggaagaagagcattgtgactgagcggcggacgggtgagtaacgcgtgggtaacctgcctcatacagggggataacagttagaaatggctgctaataccgcataagaccacagcaccgcatggtgcaggggtaaaaactccggtggtatgagatggacccgcgtctgattagctagttggtggggtaacggcctaccaaggcgacgatcagtagccgacctgagagggtgaccggccacattgggactgagacacggcccaaactcctacgggaggcagcagtggggaatattgcacaatgggggaaaccctgatgcagcgacgccgcgtgagcgaagaagtatttcggtatgtaaagctctatcagcagggaagaaaatgacggtacctgactaagaagccccggctaactacgtgccagcagccgcggtaatacgtagggggcaagcgttatccggatttactgggtgtaaagggagcgtagacggcgaggcaagtctgatgtgaaaacccggggctcaaccccgtgactgcattggaaactgttttgcttgagtgccggagaggtaagcggaattcctagtgtagcggtgaaatgcgtagatattaggaggaacaccagtggcgaaggcggcttactggacggcaactgacgttgaggctcgaaagcgtggggagcaaacaggattagataccctggtagtccacgccgtaaacgatgaatactaggtgtcggggagcaaagctcttcggtgccgccgcaaacgcaataagtattccacctggggagtacgttcgcaagaatgaaactcaaaggaattgacggggacccgcacaagcggtggagcatgtggtttaattcgaagcaacgcgaagaaccttaccaagccttgacatcccattgacagagcatgtaatgtgctttcccttcggggcagtggtgacaggtggtgcatggttgtcgtcagctcgtgtcgtgagatgttgggttaagtcccgcaacgagcgcaacccctatcttcagtagccagcggttcggccgggcactctggagagactgccagggataacctggaggaaggtggggatgacgtcaaatcatcatgccccttatggcttgggctacacacgtgctacaatggcgtaaacaaagggaagcgagcctgcgagggggagcaaatcccaaaaataacgtctcagttcggattgtagtctgcaactcgactacatgaagctggaatcgctagtaatcgcgaatcagaatgtcgcggtgaatacgttcccgggtcttgtacacaccgcccgtcacaccatgggagtcggcaacgcccgaagccagtgacccaaccgaaaggagggagctgtcgaaggcggggccggtaactggggtgaagtcgtaacaaggta

SEQ ID NO: 12 - DNA, 1321 bp, Unknown
  16S rRNA(PAC001360_g)
gatgaacgctggcggcgtgcttaacacatgcaagtcgaacggagtaggtagcaatacttactcagtggcggacgggtgagtaacgcgtgaacaatctccctatgtcaggggaataacactaagaaattggtgctaataccgcataagaccacagaggggcatccctcaggggtaaaagatttatcggacatagatgagttcgcgtcccattaggtagttggtgaggtaacggcccaccaagccgacgatgggtagccgacctgagagggtgatcggccacattggaactgagagacggtccagactcctacgggaggcagcagtggggaatattgggcaatggagggaactctgacccagcaacgccgcgtgagtgaagaaggttttcggattgtaaaactctttaagcggggacgaagaaagtgactgtacccgcagaataagcatcggctaactacgtgccagcagccgcggtaatacgtaggatgcaagcgttatccggaatgactgggcgtaaagggtgcgtaggtggtttgccaagttggcagcgtaattccgtggcttaaccgcggaactactgccaaaactggtaggcttgagtgcggcaggggtatgtggaattcctagtgtagcggtggaatgcgtagatattaggaggaacaccggtggcgaaagcgacatactgggccgtaactgacactgaggcacgaaagcgtggggagcaaacagaaggagatcccctggtagtccacccccgtaaacgatgaataaagggagtaggaggtattgcttccttctgtgcgttcgcaaacgcattaagtattccgcctggggactacggccgcaaggttgaaactcaaagaaaatgacggggacccgcacaagcagcggagcatggggtttaatttgacgcaacgcgaaaaaccttaccagaacttgacatcgagtgaagagtcttgtaatgagactcgtcccttcggggacacgaagacaggtgttgcatggttgtcgtcagctcgtgtcgtgagatgttaggttaagtcctgcaacgagcgcaaccctcatatacagttgccaatattcagttaggaactctgtatagactgccgtggtcaacacggaggaaggtggggaggacgtcaaatcatcacggcccttacgttctgggccacacccgtgctacaatggctattacaaagagcagcgagatagtaatatggagcgaatctcagaaagatagtctcagttcagagtgtgggctgcaactcgcccacacgaagtaggagttgctagtaatcccgaatcagcatgtcggggtgaa

SEQ ID NO: 13 - DNA, 1487 bp, Unknown
  16S rRNA(Porphyromonas genus)
agagtttgactctggctcaggatgaacgctagcgataggcttaacacatgcaagtcgaggggcagcgagatgtagcaatacgtcgtcggcgaccggcgaatgggtgagtaacacgtatgcaacttacctcttagtggtgaataacccgatgaaagtcggactaatacaccatatactccttagatcccatgagaagaggaggaaagattaatcgctaagagatgggcctgcgttccattagctagttggtaaggtaacggcttaccaaggcaacgatggatagggggactgagaggttgaccccccacattgacactgagatacgggtcaaactcctacgggaggcagcagtgaggaatattggtcaatgggcgagagcctgaaccagccaagtcgcgtgaaggaagactgcccgcaagggttgtaaacttcttttgtatgggattaaagtcacctacgtgtaggtgtttgcagttaccatacgaataagcatcggctaactccgtgccagcagccgcggtaatacggaggatgcgagcgttatccggaattattgggtttaaagggtgcgtaggttgcaagggaagtcaggggtgaaaagctgtagctcaactatggtcttgcctttgaaactctctagctagagtgtactggaggtacgtggaacgtgtggtgtagcggtgaaatgcatagatatcacacagaactccgattgcgcaggcagcgtactacattacaactgacactgaagcacgaaagcgtgggtatccaacaggattagataccctggtagtccacgcagtaaacgatgaatactagatctatgcgatatacagtatgggtctaagcgaaagcgataagtattccacctggggagtacgccggcaacggtgaaactcaaagagattggcgggggtccgcacaagcggaggaacatgtggtttaattcgatgatacgcgaggaaccttacccgggattgaaatgtagatgcatgaggctgagaggtctcttcccttcggggcttctatgtaggtgctgcatggttgtcgtcagctcgtgccgtgaggtgtcggcttaagtgccataacgagcgcaacccgcgtcgatagttactaacgagtcaagtcgaggactctatcgagacagccgtcgtaagacgtgaggaaggagcggatgacgtcaaatcagcacggcccttacatccggggcgacacacgtgttacaatggtagggacagcgagcagccatctggtgacagagagctaatctataaaccctatcccagttcggatcggagtctgcaactcgactctgtgaagctggattcgctagtaatcgcgcatcagccatggcgcggtgaatacgttcccggaccttgcacacaccgcccgtcaagccatgggagtcgggggtacctgaagagcgtgaccgtcacaggagcgcttgagggtaaaactggtgactggggctaagtcgtaacaaggta

SEQ ID NO: 14 - DNA, 1486 bp, Unknown
  16S rRNA(Ruthenibacterium genus)
agagtttgatcctggctcaggacgaacgctggcggcgcgcctaacacatgcaagtcgaacggagctgttttctctgaagttttcggatggaagagagttcagcttagtggcgaacgggtgagtaacacgtgagcaacctgcctttcagtgggggacaacatttggaaacgaatgctaataccgcataagaccacagtgtcgcatggcacaggggtcaaaggatttatccgctgaaagatgggctcgcgtccgattagctagatggtgaggtaacggcccaccatggcgacgatcggtagccggactgagaggttgaacggccacattgggactgagacacggcccagactcctacgggaggcagcagtggggaatattgcacaatgggggaaaccctgatgcagcgacgccgcgtggaggaagaaggtcttcggattgtaaactcctgtcccaggggacgataatgacggtaccctgggaggaagcaccggctaactacgtgccagcagccgcggtaaaacgtagggtgcaagcgttgtccggaattactgggtgtaaagggagcgcaggcggattggcaagttgggagtgaaatctatgggctcaacccataaattgctttcaaaactgtcagtcttgagtggtgtagaggtaggcggaattcccggtgtagcggtggaatgcgtagatatcgggaggaacaccagtggcgaaggcggcctactgggcactaactgacgctgaggctcgaaagcatgggtagcaaacaggattagataccctggtagtccatgccgtaaacgatgattactaggtgtgggaggattgaccccttccgtgccgcagttaacacaataagtaatccacctggggagtacgaccgcaaggttgaaactcaaaggaattgacgggggcccgcacaagcagtggagtatgtggtttaattcgaagcaacgcgaagaaccttaccaggtcttgacatcggatgcatacctaagagattagggaagtccttcgggacatccagacaggtggtgcatggttgtcgtcagctcgtgtcgtgagatgttgggttaagtcccgcaacgagcgcaacccttatcgttagttactacgcaagaggactctagcgagactgccgttgacaaaacggaggaaggtggggatgacgtcaaatcatcatgccctttatgacctgggctacacacgtactacaatggctattaacagagagaagcgataccgcgaggtggagcaaacctcacaaaaatagtctcagttcggatcgcaggctgcaacccgcctgcgtgaagccggaattgctagtaatcgcggatcagcatgccgcggtgaatacgttcccgggccttgtacacaccgcccgtcacaccatgagagccggggggacccgaagtcggtagtctaaccgtaaggaggacgccgccgaaggtaaaactggtgattggggtgaagtcgtaacaaggta

SEQ ID NO: 15 - DNA, 1456 bp, Unknown
  16S rRNA(Acetitomaculum genus)
gatgaacgctggcggcgtgcctaacacatgcaagttgaacgaagcacttacgacggaatcctccgggaggaagatgtaagcgacttagtggcggacgggtgagtaacgcgtgggtaacctgccctgtacagggggacaacagccggaaacagctgctaataccccataagcgcacggtatcgcatgatacagtgtgaaaagccgagacggtacaggatggacccgcgtctgattagatagttggtggggtaacggcctaccaagtcagcgatcagtagccggcctgagagggtgaacggccacattggaactgagacacggtccaaactcctacgggaggcagcagtggggaatattgcacaatgggggaaaccctgatgcagcgacgccgcgtgaaggaagaagtatttcggtatgtaaacttctatcagcagggaagaaaatgacggtacctgactaagaagtcccggctaactacgtgccagcagccgcggtaatacgtagggggcaagcgttatccggatttactgggtgtaaagggagcgtaggcggcatggcaagccagatgtgaaaggccggggctcaaccccgggactgcatttggaactgtcaggcttgagtgttggagaggtaagcggaattcctagtgtagcggtgaaatgcgtagatattaggaggaacaccagtggcgaaggcggcttactggacaataactgacgctgaggctcgaaagcgtggggagcaaacaggattagataccctggtagtccacgccgtaaacgatgaatactaggtgtcggggtccgacaggactccggtgccgcagcaaacgcagtaagtattccacctggggagtacgttcgcaagaatgaaactcaaaggaattgacggggacccgcacaagcggtggagcatgtggtttaattcgaagcaacgcgaagaaccctaccaaatcttgacatcccactgacagcacatgtaaagtgtgtttccttcgggacagtggtgacaggtggtgcatggttgtcgtcagctcgtgtcgtgagatgttgggttaagtcccgcaacgagcgcaacccctgtttccagtagccagcaggcagggctgggcactctggagagactgccggggacaacccggaggaaggcggggatgacgtcaaatcatcatgccccttatgatttgggctacacacgtgctacaatggcgtaaacagagggaagcagccctgtgaaggtgagcaaatcccaaaataacgtcccagttcggattgtagtctgcaacccgactacatgaagctggaatcgctagtaatcgcagatcagaatgctgcggtgaatacattcccgggtcttgtacacaccgcccgtcacaccatgggagttggaaatgcccgaagtcagtgacccaaccgcaaggagggagctgccgaaggcaggttcgataactggggtg

SEQ ID NO: 16 - DNA, 1458 bp, Unknown
  16S rRNA(Adlercreutzia genus)
agagtttgatcctggctcaggatgaacgctggcggcgtgcttaacacatgcaagtcgaacgattaagacggcttcggccgtgtatagagtggcgaacgggtgagtaacacgtgaccaacctgccccgcgctccgggacaaccgctggaaacggcggctaataccggatgctccggggaggccccatggcctccccgggaaagccctgacggcgcgggatggggtcgcggcccattaggtagacggcggggtaacggcccaccgtgcccgcgatgggtagccggactgagaggtcgaccggccacattgggactgagatacggcccagactcctacgggaggcagcagtggggaattttgcgcaatgggggcaaccctgacgcagcaacgccgcgtgcgggacgaaggccttcgggttgtaaaccgctttcagcagggaagacatagacggtacctgcagaagaagctccggctaactacgtgccagcagccgcggtaatacgtagggggcgagcgttatccggattcattgggcgtaaagcgcgcgtaggcggccgcctaagcggaacctctaatcccggggctcaacctcgggccgggttccggactgggcggctcgagtgcggtagaggcaggcggaattcccggtgtagcggtggaatgcgcagatatcgggaagaacaccgatggcgaaggcagcctgctgggccgccactgacgctgaggcgcgaaagctgggggagcgaacaggattagataccctggtagtcccagccgtaaacgatggacgctaggtgtggggggaccatccccccgtgccgcagccaacgcattaagcgtcccgcctggggagtacggccgcaaggctaaaactcaaaggaattgacgggggcccgcacaagcagcggagcatgtggcttaattcgaagcaacgcgaagaaccttaccagggcttgacatgcgagtgaagccgcggagacgcggtggccgagaggagctcgcgcaggtggtgcatggctgtcgtcagctcgtgtcgtgagatgttgggttaagtcccgcaacgagcgcaacccccgtcccgtgttgccagcattcagttggggactcgcgggagactgccggcgtcaagccggaggaaggtggggacgacgtcaagtcatcatgccccttatgccctgggctgcacacgtgctacaatggccggtacagagggttgccaccccgcgagggggagcggatcccggaaagccggtcccagttcggatcgcaggctgcaacccgcctgcgtgaagtcggagttgctagtaatcgcggatcagcatgccgcggtgaatacgttcccgggccttgtacacaccgcccgtcacaccacccgagtcgtctgcacccgaagccgccggccgaacccttctggggcggaggcgtcgaaggtgtggagggtaaggggggtgaagtcgta

SEQ ID NO: 17 - DNA, 1383 bp, Unknown
  16S rRNA(Agathobaculum genus)
ttagtggcggacgggtgagtaacgcgtgagcaatctgcctttaagagggggataacagtcggaaacggctgctaataccgcataaagcatcaaattcgcatgtttttgatgccaaaggagcaatccgcttttagatgagctcgcgtctgattagctggttggcggggtaacggcccaccaaggcgacgatcagtagccggactgagaggttgaacggccacattgggactgagacacggcccagactcctacgggaggcagcagtggggaatattgcgcaatgggggaaaccctgacgcagcaacgccgcgtgattgaagaaggccttcgggttgtaaagatctttaatcagggacgaaacaaatgacggtacctgaagaataagctccggctaactacgtgccagcagccgcggtaatacgtagggagcaagcgttatccggatttactgggtgtaaagggcgcgcaggcgggccggcaagttggaagtgaaatctatgggcttaacccataaactgctttcaaaactgctggtcttgagtgatggagaggcaggcggaattccgtgtgtagcggtgaaatgcgtagatatacggaggaacaccagtggcgaaggcggcctgctggacattaactgacgctgaggcgcgaaagcgtggggagcaaacaggattagataccctggtagtccacgccgtaaacgatggatactaggtgtgggaggtattgaccccttccgtgccgcagttaacacaataagtatcccacctggggagtacggccgcaaggttgaaactcaaaggaattgacgggggcccgcacaagcagtggagtatgtggtttaattcgaagcaacgcgaagaaccttaccaggtcttgacatcccgatgaccgcttcagagatgagccttttcttcggaacatcggagacaggtggtgcatggttgtcgtcagctcgtgtcgtgagatgttgggttaagtcccgcaacgagcgcaacccttacggttagttgatacgcaagatcactctagccggactgccgttgacaaaacggaggaaggtggggacgacgtcaaatcatcatgccccttatgacctgggctacacacgtactacaatggcagtcatacagagggaagcaaaaccgcgaggtggagcaaatccctaaaagctgtcccagttcagattgcaggctgcaacccgcctgcatgaagtcggaattgctagtaatcgcggatcagcatgccgcggtgaatacgttcccgggccttgtacacaccgcccgtcacaccatgagagccgtcaatacccgaagtccgtagcctaaccgtaaggagggcgcggccgaaggtaggggtggtaattagggtgaagtcgtaaca

SEQ ID NO: 18 - DNA, 1485 bp, Unknown
  16S rRNA(Alistipes genus)
agagtttgatcctggctcaggatgaacgctagcggcaggcttaacacatgcaagtcgaggggcagcataatggatagcaatatctatggtggcgaccggcgcacgggtgcgtaacgcgtatgcaacctacctttaacagggggataacactgagaaattggtactaataccccataatatcatagaaggcatcttttatggttgaaaattccgatggttagagatgggcatgcgttgtattagctagttggtggggtaacggctcaccaaggcgacgatacatagggggactgagaggttaaccccccacactggtactgagacacggaccagactcctacgggaggcagcagtgaggaatattggtcaatggacgcaagtctgaaccagccatgccgcgtgcaggatgacggctctatgagttgtaaactgcttttgtacgagggtaaacgcagatacgtgtatctgtctgaaagtatcgtacgaataaggatcggctaactccgtgccagcagccgcggtaatacggaggattcaagcgttatccggatttattgggtttaaagggtgcgtaggcggtttgataagttagaggtgaaatttcggggctcaaccctgaacgtgcctctaatactgttgagctagagagtagttgcggtaggcggaatgtatggtgtagcggtgaaatgcttagagatcatacagaacaccgattgcgaaggcagcttaccaaactatatctgacgttgaggcacgaaagcgtggggagcaaacaggattagataccctggtagtccacgcagtaaacgatgataactcgttgtcggcgatacacagtcggtgactaagcgaaagcgataagttatccacctggggagtacgttcgcaagaatgaaactcaaaggaattgacgggggcccgcacaagcggaggaacatgtggtttaattcgatgatacgcgaggaaccttacccgggcttgaaagttagcgacgattcttgaaagaggatttcccttcggggcgcgaaactaggtgctgcatggttgtcgtcagctcgtgccgtgaggtgtcgggttaagtcccataacgagcgcaacccctaccgttagttgccatcaggtgaagctgggcactctggcgggactgccggtgtaagccgagaggaaggtggggatgacgtcaaatcagcacggcccttacgtccggggctacacacgtgttacaatggtaggtacagagggcagctacccagcgatgggatgcgaatctcgaaagcctatctcagttcggattggaggctgaaacccgcctccatgaagttggattcgctagtaatcgcgcatcagccatggcgcggtgaatacgttcccgggccttgtacacaccgcccgtcaagccatgggagccgggggtgcctgaagttcgtgaccgcaaggagcgacctagggcaaaactggtgactggggctaagtcgtaacaaggta

SEQ ID NO: 19 - DNA, 1487 bp, Unknown
  16S rRNA(Anaerostipes genus)
tttgatcctggctcaggatgaacgctggcggcgtgcttaacacatgcaagtcgaacgaaacaccttatttgattttcttcggaactgaagatttggtgattgagtggcggacgggtgagtaacgcgtgggtaacctgccctgtacagggggataacagtcagaaatgactgctaataccgcataagaccacagcaccgcatggtgcaggggtaaaaactccggtggtacaggatggacccgcgtctgattagctggttggtgaggtaacggctcaccaaggcgacgatcagtagccggcttgagagagtgaacggccacattgggactgagacacggcccaaactcctacgggaggcagcagtggggaatattgcacaatgggggaaaccctgatgcagcgacgccgcgtgagtgaagaagtatctcggtatgtaaagctctatcagcagggaagaaaatgacggtacctgactaagaagccccggctaactacgtgccagcagccgcggtaatacgtagggggcaagcgttatccggaattactgggtgtaaagggtgcgtaggtggtatggcaagtcagaagtgaaaacccagggcttaactctgggactgcttttgaaactgtcagactggagtgcaggagaggtaagcggaattcctagtgtagcggtgaaatgcgtagatattaggaggaacatcagtggcgaaggcggcttactggactgaaactgacactgaggcacgaaagcgtggggagcaaacaggattagataccctggtagtccacgccgtaaacgatgaatactaggtgtcggggccgtaggggcttcggtgccgcagccaacgcagtaagtattccacctggggagtacgttcgcaagaatgaaactcaaaggaattgacggggacccgcacaagcggtggagcatgtggtttaattcgaagcaacgcgaagaaccttacctggtcttgacatccttctgaccggtccttaaccggacctttccttcgggacaggagagacaggtggtgcatggttgtcgtcagctcgtgtcgtgagatgttgggttaagtcccgcaacgagcgcaacccctatctttagtagccagcatataaggtgggcactctagagagactgccagggataacctggaggaaggtggggacgacgtcaaatcatcatgccccttatgaccagggctacacacgtgctacaatggcgtaaacagagggaagcagcctcgtgagagtgagcaaatcccaaaaataacgtctcagttcggattgtagtctgcaactcgactacatgaagctggaatcgctagtaatcgcgaatcagaatgtcgcggtgaatacgttcccgggtcttgtacacaccgcccgtcacaccatgggagtcagtaacgcccgaagtcagtgacccaaccgtaaggagggagctgccgaaggcgggaccgataactggggtgaagtcgtaacaaggta

SEQ ID NO: 20 - DNA, 1523 bp, Unknown
  16S rRNA(Blautia genus)
agagtttgatcctggctcaggatgaacgctggcggcgtgcttaacacatgcaagtcgaacgggaattactttattgaaacttcggtcgatttaatttaattctagtggcggacgggtgagtaacgcgtgggtaacctgccttatacagggggataacagtcagaaatggctgctaataccgcataagcgcacagagctgcatggctcagtgtgaaaaactccggtggtataagatggacccgcgttggattagctagttggtggggtaacggcccaccaaggcgacgatccatagccggcctgagagggtgaacggccacattgggactgagacacggcccagactcctacgggaggcagcagtggggaatattgcacaatgggggaaaccctgatgcagcgacgccgcgtgaaggaagaagtatctcggtatgtaaacttctatcagcagggaagatagtgacggtacctgactaagaagccccggctaactacgtgccagcagccgcggtaatacgtagggggcaagcgttatccggatttactgggtgtaaagggagcgtagacggtgtggcaagtctgatgtgaaaggcatgggctcaacctgtggactgcattggaaactgtcatacttgagtgccggaggggtaagcggaattcctagtgtagcggtgaaatgcgtagatattaggaggaacaccagtggcgaaggcggcttactggacggtaactgacgttgaggctcgaaagcgtggggagcaaacaggattagataccctggtagtccacgccgtaaacgatgaatactaggtgtcggggagcatggctcttcggtgccgtcgcaaacgcagtaagtattccacctggggagtacgttcgcaagaatgaaactcaaaggaattgacggggacccgcacaagcggtggagcatgtggtttaattcgaagcaacgcgaagaaccttaccaagtcttgacatccgcctgaccgatccttaaccggatctttccttcgggacaggcgagacaggtggtgcatggttgtcgtcagctcgtgtcgtgagatgttgggttaagtcccgcaacgagcgcaacccctatcctcagtagccagcatttaaggtgggcactctggggagactgccagggataacctggaggaaggcggggatgacgtcaaatcatcatgccccttatgatttgggctacacacgtgctacaatggcgtaaacaaagggaagcgagattgtgagatggagcaaatcccaaaaataacgtcccagttcggactgtagtctgcaacccgactacacgaagctggaatcgctagtaatcgcggatcagaatgccgcggtgaatacgttcccgggtcttgtacacaccgcccgtcacaccatgggagtcagtaacgcccgaagtcagtgacctaactgcaaagaaggagctgccgaaggcgggaccgatgactggggtgaagtcgtaacaaggtagccgtatcggaaggtgcggctggatcacctccttt

SEQ ID NO: 21 - DNA, 1399 bp, Unknown
  16S rRNA(CCMM_g)
tggctcaggatgaacgctggcggcgtgcctaatacatgcaagtcgaacgcttcacatatgtgaagagtggcgaacgggtgagtaatacataagtaacctggcctttacagggggataactgttggaaacgatagctaagaccgcataggtgtcataaccgcatggagatgatatgaaatatgctacggcataggtagaggatggacttatggcgcattagctagttggaggggtaacggcccaccaaggcgacgatgcgtagccgacctgagagggtgaccggccacactgggactgagacacggcccagactcctacgggaggcagcagtagggaattttcggcaatgggggaaaccctgaccgagcaacgccgcgtgaaggaagaagtaattcgttatgtaaacttctgtcatagaggaagaacggtgcgtgtagggaatgacatgcaagtgacggtactctataagaaagccacggctaactacgtgccagcagccgcggtaatacgtaggtggcgagcgttatccggaattattgggcgtaaagagggagcaggcggcactaagggtctgtggtgaaagatcgaagcttaacttcggtaagccatggaaaccgtagagctagagtgtgtgagaggatcgtggaattccatgtgtagcggtgaaatgcgtagatatatggaggaacaccagtggcgaaggcgacgatctggcgcataactgacgctcagtcccgaaagcgtggggagcaaataggattagataccctagtagtccacgccgtaaacgatgagtactaagtgttgggagtcaaatctcagtgctgcagttaacgcaataagtactccgcctgagtagtacgttcgcaagaatgaaactcaaaggaattgacgggggcccgcacaagcggtggagcatgtggtttaattcgaagcaacgcgaagaaccttaccaggtcttgacatcgatctaaaggctccagagatggagagatagctatagagaagacaggtggtgcatggttgtcgtcagctcgtgtcgtgagatgttgggttaagtcccgcaacgagcgcaacccctgttgccagttgccagcattaagttggggactctggcgagactgccggtgacaagccggaggaaggcggggatgacgtcaaatcatcatgccccttatgacctgggctacacacgtgctacaatggacagagcagagggaagcgaagccgcgaggtggagcgaaacccagaaaactgttctcagttcggactgcagtctgcaactcgactgcacgaagttggaatcgctagtaatcgcgaatcagcatgtcgcggtgaatacgttctcgggccttgtacacaccgcccgtcacaccatgagagtcggtaacacccgaag

SEQ ID NO: 22 - DNA, 1453 bp, Unknown
  16S rRNA(Christensenella genus)
gacgaacgctggcggcgtgcttaacacatgcaagtcgaacgaagcagcttaacggaactcttcggagggcagatgagttgactgagtggcggacgggtgagtaacgcgtgagcaacctgcccataagagggggataacagttggaaacgactgctaataccgcataagaccacattaccgcatggtagagaggtcaaagaaattcgcttatggaggggctcgcgtcccattaggtagttggtagggtaaaggcctaccaagccgacgatgggtagccgacctgagagggtgatcggccacactgaactgagacacggtccagactcctacgggaggcagcagtggggaatattgggcaatgggcgcaagcctgacccagcaacgccgcgtgagggaagaaggccttcgggttgtaaacctctgtcctatgggaagaagaaagcgacggtaccataggaggaagctccggctaactacgtgccagcagccgcggtaatacgtagggagcaagcgttgtccggaattactgggcgtaaagggtgcgtaggcggttgtttaagtcagatgtgaaatacccgggcttaactcgggggctgcatctgatactggataactagagtgcaggagaggaaagtggaattcctagtgtagcggtggaatgcgtagatattaggaggaacaccagtggcgaaggcgactttctggactgtaactgacgctgaggcacgaaagtatgggtagcaaacaggattagataccctggtagtccatactgtaaacgatgaatactaggtgtgggggacaatagtcttccgtgccgcagccaacgcaataagtattccgcctggggagtacggtcgcaagactgaaactcaaaggaattgacgggggcccgcacaagcagcggagcatgtggtttaattcgaagcaacgcgaagaaccttaccaaggcttgacatcccggtgaccggcatagagatatgccttctcttcggagcaccggtgacaggtggtgcatggttgtcgtcagctcgtgtcgtgagatgttgggttaagtcccgcaacgagcgcaacccttgttactagttgccagcatttcggatgggaactctagtgagactgccggggataactcggaggaaggtggggatgacgtcaaatcatcatgccctttatgtcttgggctacacacgtgctacaatggtcggtacaaagagcggcgagctcgtaagagtaagcgaatctcataaagccggtctcagttcagattgtgggctgcaacccgcccacatgaagtcggagttgctagtaatcgcggatcagcatgccgcggtgaatgcgttcccgggccttgtacacaccgcccgtcacaccatggaagttgggggcgcccgaagccgatggcctaaccgcaaggagggagtcgtcgaaggtgaaaccaatgactggggtg

SEQ ID NO: 23 - DNA, 1476 bp, Unknown
  16S rRNA(Coprococcus genus)
agagtttgatcctggctcaggatgaacgctggcggcgtgcttaacacatgcaagtcgaacgattgaagctggagcttgctccggccgatttagtggcggacgggtgagtaacgcgtgggtaacctgcctcatacagggggatagcagttggaaacgactggtaaaaccgcataagcgcacggtatcgcatgatacagtgtgaaaacactccggtggtatgagatggacccgcgtctgattagctagttggtgaggtaacggcccaccaaggcgacgatcagtagccggcctgagagggtgaacggccacattgggactgagacacggcccaaactcctacgggaggcagcagtggggaatattgcacaatgggggaaaccctgatgcagcgacgccgcgtgagtgaagaagtatttcggtatgtaaagctctatcagcagggaagataatgacggtacctgactaagaagcaccggctaaatacgtgccagcagccgcggtaatacgtatggtgcaagcgttatccggatttactgggtgtaaagggtgcgtaggtggcaaggcaagtctgaagtgaaaatccggggctcaaccccggaactgctttggaaactgtttagctagagtacaggagaggtaagtggaattcctagtgtagcggtgaaatgcgtagatattaggaggaacaccagtggcgaaggcgacttactggactgctactgacactgaggcacgaaagcgtggggagcaaacaggattagataccctggtagtccacgccgtaaacgatgaatactaggtgttgggttccaaagggactcggtgccgtcgcaaacgcattaagtattccacctggggagtacgttcgcaagaatgaaactcaaaggaattgacggggacccgcacaagcggtggagcatgtggtttaattcgaagcaacgcgaaaaaccttaccaagtcttgacatcctgatgacagtttcttaaccggaacttctcttcggagcatcagagacaggtggtgcatggttgtcgtcagctcgtgtcgtgagatgttgggttaagtcccgcaacgagcgcaacccctatttccagtagccagcagtaagatgggcactctggagagactgccggggataacccggaggaaggtggggatgacgtcaaatcatcatgccccttatgatttgggctacacacgtgctacaatggcagttacaaagagaagcaaacctgtgaaggcgagcaaacctcaaaaaggctgtctcagttcggattgtagtctgcaactcgactacatgaagctggaatcgctagtaatcgcagatcagcatgctgcggtgaatacgttcccgggtcttgtacacaccgcccgtcacaccatgggagtcggtaacgcccgaagtcagtgacccaaccgcaaggagggagctgccgaaggcaggatcgataactggggtgaagtcgtaacaaggta

SEQ ID NO: 24 - DNA, 1469 bp, Unknown
  16S rRNA(Eubacterium_g17)
gatgaacgctggcggcgtgcttaacacatgcaagtcgaacgaagcacctctcccgaagattgacacagcttgctgtagattgattcatttgaggtgactgagtggcggacgggtgagtaacgcgtgggtaacctgcctcatagagggggacaacagttggaaacgactgctaataccgcatagtaagaaagattcgcatgtttctttcttgaaagatttatcgctatgagatggacccgcgtctgattagctagttggtaaggtaacggcttaccaaggcgacgatcagtagccggcttgagagagtgaacggccacattgggactgagacacggcccaaactcctacgggaggcagcagtggggaatattgcacaatgggggaaaccctgatgcagcgacgccgcgtgagtgaagaagtatttcggtatgtaaagctctatcagcagggaagataatgacggtacctgactaagaagccccggctaactacgtgccagcagccgcggtaatacgtagggggcaagcgttatccggatttactgggtgtaaagggtgcgtaggtggcaaggcaagtcagatgtgaaagcccggggctcaaccccggtactgcatttgaaactgtctagctagagtgcaggagaggtaagcggaattcctagtgtagcggtgaaatgcgtagatattaggaggaacaccagtggcgaaggcggcttactggactgtaactgacactgaggcacgaaagcgtggggagcaaacaggattagataccctggtagtccacgccgtaaacgatgaatactaggtgtcggggcccacagggcttcggtgccgcagcaaacgcattaagtattccacctggggagtacgttcgcaagaatgaaactcaaaggaattgacggggacccgcacaagcggtggagcatgtggtttaattcgaagcaacgcgaagaaccttaccaagtcttgacatccttctgaccgttccttagccggaacttctcttcggagcagaagtgacaggtggtgcatggttgtcgtcagctcgtgtcgtgagatgttgggttaagtcccgcaacgagcgcaacccttatccttagtagccagcggttcggccgggcactctggggagactgccggagataatccggaggaaggtggggatgacgtcaaatcatcatgccccttatgacttgggctacacacgtgctacaatggcggtaacaaagggaagcagcctcgcgagagtgagcaaaccccaaaaatgccgtctcagttcggattgtagtctgcaactcgactacatgaagctggaatcgctagtaatcgcagatcagaatgctgcggtgaatacgttcccgggtcttgtacacaccgcccgtcacaccatgggagtcggatatgcccgaagccagtgacccaaccgcaaggagggagctgtcgaaggtggagccgataactggggtg

SEQ ID NO: 25 - DNA, 1493 bp, Unknown
  16S rRNA(Eubacterium_g20)
agagtttgatcctggctcaggatgaacgctggcggcgtgcttaacacatgcaagtcgaacgaagcactttattacgatttcttcggaatgacgatttagtgactgagtggcggacgggtgagtaacgcgtgggtaacctgccttatacagggggataacagttagaaatgactgctaataccgcataagcgcacaggattgcatgatctggtgtgaaaaactccggtggtataagatggacccgcgtctgattagctggttggtgaggtaacggcccaccaaggcgacgatcagtagccgacctgagagggtgaccggccacattgggactgagacacggcccaaactcctacgggaggcagcagtggggaatattgcacaatgggggaaaccctgatgcagcgacgccgcgtgagcgaagaagtatttcggtatgtaaagctctatcagcagggaagaaaaaaatgacggtacctgactaagaagccccggctaactacgtgccagcagccgcggtaatacgtagggggcaagcgttatccggatttactgggtgtaaagggagcgcaggcggtgcggcaagtctgatgtgaaagcccggggctcaaccccgggactgcattggaaactgtcgtacttgagtatcggagaggtaagtggaattcctagtgtagcggtgaaatgcgtagatattaggaggaacaccagtggcgaaggcggcttactggacgataactgacgctgaggctcgaaagcgtggggagcaaacaggattagataccctggtagtccacgccgtaaacgatgaatactaggtgtcgggggacatagtccttcggtgccgcagcaaacgcaataagtattccacctggggagtacgttcgcaagaatgaaactcaaaggaattgacggggacccgcacaagcggtggagcatgtggtttaattcgaagcaacgcgaagaaccttaccaagtcttgacatcccggtgacaaagtatgtaatgtactctttcttcggaacaccggtgacaggtggtgcatggttgtcgtcagctcgtgtcgtgagatgttgggttaagtcccgcaacgagcgcaacccctgtccttagtagccagcggttcggccgggcactctagggagactgccagggataacctggaggaaggcggggatgacgtcaaatcatcatgccccttatgacttgggctacacacgtgctacaatggcgtaaacaaagggaagcgaaaaggtgacttctagcaaatcccaaaaataacgtcccagttcggactgtagtctgcaactcgactacacgaagctggaatcgctagtaatcgcgaatcagaatgtcgcggtgaatacgttcccgggtcttgtacacaccgcccgtcacaccatgggagtcgggaatgcccgaagccggtgactcaaccgtaaggagagagccgtcgaaggcaggtctgataactggggtgaagtcgtaacaaggta

SEQ ID NO: 26 - DNA, 1454 bp, Unknown
  16S rRNA(Eubacterium_g23)
gatgaacgctggcggcgtgcctaacacatgcaagtcgaacgaagcttgacggatgatttcttcggaatgaaaccagatatgacttagtggcggacgggtgagtaacacgtgagcaacctgcctttcagagggggataacggctggaaacggtcgctaataccgcatgatgtgttcggatggcatcatctgaacatcaaagatttatcgctgaaagatgggctcgcgtctgattagatagttggtggggtaacggcctaccaagtcgacgatcagtagccggactgagaggttgaacggccacattgggactgagatacggcccagactcctacgggaggcagcagtggggaatattgcacaatgggggaaaccctgatgcagcaacgccgcgtgaaggatgacggttttcggattgtaaacttcttttcttagtgacgaagacagtgacggtagctaaggaataagcatcggctaactacgtgccagcagccgcggtaatacgtaggatgcaagcgttatccggatttactgggtgtaaagggagcgcaggcgggactgcaagttggatgtgaaataccgtggcttaaccacggaactgcatccaaaactgtagttcttgagtgaagtagaggcaagcggaattccgagtgtagcggtgaaatgcgtagatattcggaggaacaccagtggcgaaggcggcttgctgggctttaactgacgctgaggctcgaaagtgtggggagcaaacaggattagataccctggtagtccacactgtaaacgatgatagctaggtgtggggggtctgaccccttccgtgccggagttaacgcaataagctatccacctggggagtacgaccgcaaggttgaaactcaaaggaattgacgggggcccgcacaagcagtggattatgtggtttaattcgaagcaacgcgaagaaccttaccaggtcttgacatccgactaacgagatagagatatgtcaggtgcccttcggggaaagtcgagacaggtggtgcatggttgtcgtcagctcgtgtcgtgagatgttgggttaagtcccgcaacgagcgcaacccctgccattagttgctacgcaagagcactctaatgggaccgctaccgacaaggtggaggaaggtggggacgacgtcaaatcatcatgccccttatgacctgggctacacacgtaatacaatggccgttaacagagggaagcaaagcggtgacgcagagcaaaaccctaaaaacggtcccagttcggactgtaggctgcaacccgcctacacgaagttggaattgctagtaatcgcggatcagcatgccgcggtgaatacgttcccgggccttgtacacaccgcccgtcacaccatgggagtttgtaacacccgaagtcagtgacccaaccgcaaggagggagctgccgaaggtgggataagcgactggggtg

SEQ ID NO: 27 - DNA, 1479 bp, Unknown
  16S rRNA(Eubacterium_g24)
agagtttgatcctggctcaggatgaacgctggcggcgtgcttaacacatgcaagtcgaacgaagatgccggagtgcttgcactttggcagactgagtggcggacgggtgagtaacgcgtgggtaacctgccttatacagggggataacagttggaaacgactgctaataccgcataagcgcacggtatcgcatgatacagtgtgaaaaactccggtggtataagatggacccgcgtctgattagcttgttggtgaggtaacggcccaccaaggcgacgatcagtagccggcctgagagggtgaacggccacattgggactgagacacggcccaaactcctacgggaggcagcagtggggaatattgcacaatgggggaaaccctgatgcagcgacgccgcgtgagtgatgaagtatttcggtatgtaaaactctatcagcagggaagataatgacggtacctgactaagaagcaccggctaaatacgtgccagcagccgcggtaatacgtatggtgcaagcgttatccggatttactgggtgtaaagggtgcgtaggtggtatggcaagtcagaagtgaaaggctggggctcaaccccgggactgcttttgaaactgtcaaactagagtacaggagaggaaagcggaattcctagtgtagcggtgaaatgcgtagatattaggaggaacaccagtggcgaaggcggctttctggactgaaactgacactgaggcacgaaagcgtggggagcaaacaggattagataccctggtagtccacgccgtaaacgatgaatactaggtgtcgggcagcatagctgttcggtgccgcagcaaacgcattaagtattccacctggggagtacgttcgcaagaatgaaactcaaaggaattgacggggacccgcacaagcggtggagcatgtggtttaattcgaagcaacgcgaagaaccttaccaggtcttgacatcccgatggccgcttcttaatcgaagcttttcttcggaacatcggagacaggtggtgcatggttgtcgtcagctcgtgtcgtgagatgttgggttaagtcccgcaacgagcgcaacccctattttcagtagccagcattttggatgggcactctggagagactgcccgggataaccgggaggaaggtggggatgacgtcaaatcatcatgccccttatgatctgggctacacacgtgctacaatggctgttacagagagaagcgaatccgcgaggaagagcaaacctcaaaaaggcagtctcagttcggattgtagtctgcaactcgactacatgaagctggaatcgctagtaatcgcgaatcagaatgtcgcggtgaatacgttcccgggtcttgtacacaccgcccgtcacaccatgggagttggaaatgcccgaagtcagtgacccaaccgcaaggagggagctgccgaaggcaggttcgatgactggggtgaagtcgtaacaaggta

SEQ ID NO: 28 - DNA, 1461 bp, Unknown
  16S rRNA(Faecalibacterium genus)
gatcctggctcaggcgaacgctggcggcgcgcctaacacatgcaagtcgaacgagcgagagagagcttgctttctcaagcgagtggcgaacgggtgagtaacgcgtgaggaacctgcctcaaagagggggacaacagttggaaacgactgctaataccgcataagcccacgacccggcatcgggtagagggaaaaggagcaatccgctttgagatggcctcgcgtccgattagctagttggtgaggtaacggcccaccaaggcgacgatcggtagccggactgagaggttgaacggccacattgggactgagacacggcccagactcctacgggaggcagcagtggggaatattgcacaatgggggaaaccctgatgcagcgacgccgcgtggaggaagaaggtcttcggattgtaaactcctgttgttgaggaagataatgacggtactcaacaaggaagtgacggctaactacgtgccagcagccgcggtaaaacgtaggtcacaagcgttgtccggaattactgggtgtaaagggagcgcaggcgggaaggcaagttggaagtgaaatccatgggctcaacccatgaactgctttcaaaactgtttttcttgagtagtgcagaggtaggcggaattcccggtgtagcggtggaatgcgtagatatcgggaggaacaccagtggcgaaggcggcctactgggcaccaactgacgctgaggctcgaaagtgtgggtagcaaacaggattagataccctggtagtccacactgtggccgatgtttactaggtgttggaggattgaccccttcagtgccgcagttaacacaataagtaatccacctggggagtacgaccgcaaggttgaaactcaaaggaattgacgggggcccgcacaagcagtggagtatgtggtttaattcgacgcaacgcgaagaaccttaccaagtcttgacatcctgcgacgcacatagaaatatgtgtttccttcgggacgcagagacaggtggtgcatggttgtcgtcagctcgtgtcgtgagatgttgggttaagtcccgcaacgagcgcaacccttatggtcagttactacgcaagaggactctggccagactgccgttgacaaaacggaggaaggtggggatgacgtcaaatcatcatgccctttatgacttgggctacacacgtactacaatggcgttaaacaaagagaagcaagaccgcgaggtggagcaaaactcagaaacaacgtcccagttcggactgcaggctgcaactcgcctgcacgaagtcggaattgctagtaatcgcagatcagcatgctgcggtgaatacgttcccgggccttgtacacaccgcccgtcacaccatgagagccggggggacccgaagtcggtagtctaaccgcaaggaggacgccgccgaaggtaaaactggtgattggggtgaagtcgtaacaaggta

SEQ ID NO: 29 - DNA, 1463 bp, Unknown
  16S rRNA(Frisingicoccus genus)
tggctcaggatgaacgctggcggcgcgcctaacacatgcaagtcgaacggacgatgaagagcttgcttttcaaagttagtggcggacgggtgagtaacgcgtgggtaacctgcctcatacaggggaatagcagctggaaacggctgataaaaccgcataagcgcacagtgccgcatggcacagtgtgaaaaactccggtggtatgagatggacccgcgtctgattagcttgttggcggggtaacggcccaccaaggcgacgatcagtagccggcctgagagggtgatcggccacattgggactgagacacggcccaaactcctacgggaggcagcagtggggaatattgcacaatgggggaaaccctgatgcagcgacgccgcgtgaaggaagaagtatctcggtatgtaaacttctatcagcagggaagataatgacggtacctgactaagaagccccggctaactacgtgccagcagccgcggtaatacgtagggggcaagcgttatccggatttactgggtgtaaagggagcgtaggcggcggagcaagtcagaagtgaaagcccggggctcaaccccgggacggcttttgaaactgccctgcttgatttcaggagaggtaagcggaattcctagtgtagcggtgaaatgcgtagatattaggaggaacaccagtggcgaaggcggcttactggactgacaatgacgctgaggctcgaaagcgtggggagcaaacaggattagataccctggtagtccacgccgtaaacgatgaatactaggtgtcggggctcataagagcttcggtgccgcagcaaacgcaataagtattccacctggggagtacgttcgcaagaatgaaactcaaaggaattgacggggacccgcacaagcggtggagcatgtggtttaattcgaagcaacgcgaagaaccttaccaggccttgacatcccggtgaccgacccgtaatggggtcttctctacggagcactggagacaggtggtgcatggttgtcgtcagctcgtgtcgtgagatgttgggttaagtcccgcaacgagcgcaacccctatgttcagtagccagcatttaggatgggcactctggacagactgccggggataacccggaggaaggcggggatgacgtcaaatcatcatgccccttacggcctgggctacacacgtgctacaatggcgtaaacaaagggaagcaagagggtgacctggagcgaatcccataaataacgtcccagttcggactgtagtctgcaacccgactacacgaagctggaatcgctagtaatcgcgaatcagcatgtcgcggtgaatacgttcccgggtcttgtacacaccgcccgtcacaccatgggagttggaaatgcccgaagtcagtgacctgaccgcaaggagggagctgccgaaggtggagccgatgactggggtgaagtcgtaacaaggta

SEQ ID NO: 30 - DNA, 1489 bp, Unknown
  16S rRNA(Lachnospira genus)
agagtttgatcctggctcaggatgaacgctggcggcgtgcttaacacatgcaagtcgaacgaagcatttgcgacagattttttcggaatgaagttgcttatgactgagtggcggacgggtgagtaacgcgtgggtaacctgccttgtactgggggatagcagctggaaacggctggtaataccgcataagcgcacaatgttgcatgacatggtgtgaaaaactccggtggtataagatggacccgcgtctgattagctagttggtgagataacagcccaccaaggcgacgatcagtagccgacctgagagggtgaccggccacattgggactgagacacggcccagactcctacgggaggcagcagtggggaatattgcacaatggaggaaactctgatgcagcgacgccgcgtgagtgaagaagtaattcgttatgtaaagctctatcagcagggaagatagtgacggtacctgactaagaagctccggctaaatacgtgccagcagccgcggtaatacgtatggagcaagcgttatccggatttactgggtgtaaagggagtgtaggtggccatgcaagtcagaagtgaaaatccggggctcaaccccggaactgcttttgaaactgtaaggctggagtgcaggaggggtgagtggaattcctagtgtagcggtgaaatgcgtagatattaggaggaacaccagtggcgaaggcggctcactggactgtaactgacactgaggctcgaaagcgtggggagcaaacaggattagataccctggtagtccacgccgtaaacgatgaatactaggtgtcggggcccataagggcttcggtgccgcagcaaacgcaataagtattccacctggggagtacgttcgcaagaatgaaactcaaaggaattgacggggacccgcacaagcggtggagcatgtggtttaattcgaagcaacgcgaagaaccttaccaagtcttgacatcccactgaccggacagtaatgtgtcctttccttcgggacagtggagacaggtggtgcatggttgtcgtcagctcgtgtcgtgagatgttgggttaagtcccgcaacgagcgcaacccctatccttagtagccagcagtaagatgggcactctagggagactgccagggataacctggaggaaggtggggatgacgtcaaatcatcatgccccttatgacttgggctacacacgtgctacaatggcgtaaacaaagtgaagcgaagtcgtgaggccaagcaaatcacaaaaataacgtctcagttcggattgtagtctgcaactcgactacatgaagctggaatcgctagtaatcgcagatcagaatgctgcggtgaatacgttcccgggtcttgtacacaccgcccgtcacaccatgggagtcgaaaatgcccgaagtcggtgacctaacgtaagaaggagccgccgaaggcaggtttgataactggggtgaagtcgtaacaaggta

SEQ ID NO: 31 - DNA, 1485 bp, Unknown
  16S rRNA(Lachnospiraceae_uc)
tttgatcctggctcaggatgaacgctggcggcgtgcttaacacatgcaagtcgaacgaagcaacwtatcacgattccttcgggatgacgatttgttgactgagtggcggacgggtgagtaacgcgtgggtaacctgccttatacagggggatagcagctggaaacggctgataataccgcataagcgcacggcatcgcatgatgcagtgtgaaaaactccggtggtataagatggacccgcgtctgattagctagttggtgaggtaacggcccaccaaggcaacgatcagtagccgacctgagagggtgaccggccacattgggactgagacacggcccagactcctacgggaggcagcagtggggaatattgcacaatggaggaaactctgatgcagcgacgccgcgtgagcgaagaagtatttcggtatgtaaagctctatcagcagggaagataatgacggtacctgactaagaagctccggctaaatacgtgccagcagccgcggtaatacgtatggagcaagcgttatccggatttactgggtgtaaagggagtgtaggtggcaaagcaagtcagtagtgaaaatccggggctcaacctcggaactgctattgaaactgtttagctagagtgcaggagaggtaagtggaattcctagtgtagcggtgaaatgcgtagatattaggaggaacaccagtggcgaaggcggcttactggactgtaactgacactgaggctcgaaagcgtggggagcaaacaggattagataccctggtagtccacgccgtaaacgatgaatactaggtgttgggtctcataagagattcggtgccgcagctaacgcaataagtattccacctggggagtacgttcgcaagaatgaaactcaaaggaattgacggggacccgcacaagcggtggagcatgtggtttaattcgaagcaacgcgaagaaccttacctagtcttgacatcccgatgaccragtatgtaatgtactctttcttcggaacatcggtgacaggtggtgcatggttgtcgtcagctcgtgtcgtgagatgttgggttaagtcccgcaacgagcgcaacccctatttctagtagccagcagttcggctgggcactctagagagactgccagggataacctggaggaaggtggggatgacgtcaaatcatcatgccccttatgactagggctacacacgtgctacaatggcgtaaacaaagtgaagcgagagtgtgagcttaagcaaatcacaaaaataacgtctcagttcggattgtagtctgcaactcgactacatgaagctggaatcgctagtaatcgcagatcagaatgctgcggtgaatacgttcccgggtcttgtacacaccgcccgtcacaccatgggagtcgaaaatgcccgaagtcggtgacctaacgtaagaaggagccgccgaaggcaggtttgataactggggtgaagtcgtaacaaggta

SEQ ID NO: 32 - DNA, 1432 bp, Unknown
  16S rRNA(LT821227_g)
gatgaacgctggcggcgtgcttaacacatgcaagtcgaacgattaacccaaacttcggtttggttataaagtggcgaacgggtgagtaacacgtgaccaacctgccttctagatcgggataactcaaggaaacttgtgctaataccggatactccgagaacaacgcatgttgtactcgggaaagcttttgcgctagaagatggggtcgcggcctattaggtagttggtggggtaacggcctaccaagcctgcgataggtagccgggttgagagactgatcggccacattgggactgagatacggcccagactcctacgggaggcagcagtggggaattttgcgcaatgggggcaaccctgacgcagcaacgccgcgtgcgggatgaaggtcttcggattgtaaaccgctttcagtagggaataagtttgaaggtacctacagaagaagcaccggctaaatacgtgccagcagccgcggtaatacgtatggtgcaagcgttatccggaatcattgggcgtaaagcgcgcgtaggcggcttgttaagcaggaatttaaatcttagggctcaaccttaagtcggttcctgaactggcaggctcgagtgcggtagaggaaggtggaattcccagtgtagcggtgaaatgcgcagatattgggaagaacaccgatggcgaaggcagccttctgggccgccactgacgctgaggcgcgaaagctaggggagcgaacaggattagataccctggtagtcctagccgtaaacgatgggcactaggtgtggggagttattactttccgtgccgcagctaacgcattaagtgccccgcctggggagtacggccgcaaggctaaaactcaaaggaattgacgggggcccgcacaagcagcggagcgtgtggcttaattcgaagcaacgcgaagaaccttaccagggcttgacatataggtgagctcgtggaaacacgagggccgaaaggagcctatacaggtggtgcatggctgtcgtcagctcgtgtcgtgagatgttgggttaagtcccgcaacgagcgcaacccctgttgtatgttgccagcattaagttggggactcatacaagactgccggcgtcaagccggaggaaggtggggatgacgtcaagtcatcatgccccttatgccctgggctgcacacgtgctacaatggctggtacaacgagctgcgaagtcgcgagaccaagcgaatctcttaaaaccagtcccagttcggattgcaggctgcaattcgcctgcatgaagtcggagttgctagtaatcgcggatcagcatgccgcggtgaatacgttcccgggccttgtacacaccgcccgtcacaccactcgagtcgtctgcacccgaagtcgctggcctaaccatttggaaggaggcgccgaaggtgtggagggtaagaggggtg

SEQ ID NO: 33 - DNA, 1489 bp, Unknown
  16S rRNA(Oscillibacter genus)
agagtttgatcctggctcaggacgaacgctggcggcgtgcttaacacatgcaagtcgaacgagaatctactgaaagagttttcggacaatggatgtagaggaaagtggcggacgggtgagtaacgcgtgaggaacctgccttgaagagggggacaacagttggaaacgactgctaataccgcatgatgcataggggtcgcatgatctttatgccaaagatttatcgcttcaagatggcctcgcgtctgattagctagttggcggggtaacggcccaccaaggcgacgatcagtagccggactgagaggttgaacggccacattgggactgagatacggcccagactcctacgggaggcagcagtggggaatattgggcaatgggcgcaagcctgacccagcaacgccgcgtgaaggaagaaggctttcgggttgtaaacttcttttaagagggaagagcagaagacggtacctctagaataagccacggctaactacgtgccagcagccgcggtaatacgtaggtggcaagcgttgtccggatttactgggtgtaaagggcgtgcagccgggtctgcaagtcagatgtgaaatccatgggctcaacccatgaactgcatttgaaactgtagatcttgagtgtcggaggggcaatcggaattcctagtgtagcggtgaaatgcgtagatattaggaggaacaccagtggcgaaggcggattgctggacgataactgacggtgaggcgcgaaagtgtggggagcaaacaggattagataccctggtagtccacactgtaaacgatgaatactaggtgtgcggggactgaccccctgcgtgccgcagtaaacacaataagtattccacctggggagtacgatcgcaaggttgaaactcaaaggaattgacgggggcccgcacaagcggtggattatgtggtttaattcgaagcaacgcgaagaaccttaccagggtttgacatcctgctaacgaagtagagatacattaggtgcccttcggggaaagcagagacaggtggtgcatggttgtcgtcagctcgtgtcgtgagatgttgggttaagtcccgcaacgagcgcaacccctattgttagttgctacgcaagagcactctagcgagactgccgttgacaaaacggaggaaggtggggacgacgtcaaatcatcatgccccttatatcctgggctacacacgtaatacaatggcggtcaacagagggaagcaaagccgcgaggcagagcaaacccccaaaagccgtcccagttcggattgtaggctgcaactcgcctgcatgaagtcggaatcgctagtaatcgcggatcagcatgccgcggtgaatacgttcccgggccttgtacacaccgcccgtcacaccatgagagtcgggaacacccgaagtccgtagcctaacctgaaaaggagggcgcggccgaaggtgggttcgataattggggtgaagtcgtaacaaggta

SEQ ID NO: 34 - DNA, 1489 bp, Unknown
  16S rRNA(PAC000194_g)
agagtttgatcctggctcaggatgaacgctggcggcgtgcttaacacatgcaagtcgaacgaagcacttaagtttgattcttcggatgaagacttttgtgactgagtggcggacgggtgagtaacgcgtgggtaacctgcctcatacagggggataacagttagaaatgactgctaataccgcataagaccacagcaccgcatggtgcaggggtaaaaactccggtggtatgagatggacccgcgtctgattagctagttggtggggtaacggcctaccaaggcgacgatcagtagccgacctgagagggtgaccggccacattgggactgagacacggcccaaactcctacgggaggcagcagtggggaatattgcacaatgggggaaaccctgatgcagcgacgccgcgtgaaggatgaagtatttcggtatgtaaacttctatcagcagggaagaaaatgacggtacctgactaagaagccccggctaactacgtgccagcagccgcggtaatacgtagggggcaagcgttatccggatttactgggtgtaaagggagcgtagacggtatggcaagtctgatgtgaaaggccagggctcaaccctgggactgcattggaaactgtcgaactagagtgtcggagaggcaagtggaattcctagtgtagcggtgaaatgcgtagatattaggaggaacaccagtggcgaaggcggcttgctggacgatgactgacgttgaggctcgaaagcgtggggagcaaacaggattagataccctggtagtccacgccgtaaacgatgactactaggtgtcgggtagcagagctattcggtgccgcagccaacgcaataagtagtccacctggggagtacgttcgcaagaatgaaactcaaaggaattgacggggacccgcacaagcggtggagcatgtggtttaattcgaagcaacgcgaagaaccttacctgctcttgacatctccctgaccggcaagtaatgttgcctttccttcgggacagggatgacaggtggtgcatggttgtcgtcagctcgtgtcgtgagatgttgggttaagtcccgcaacgagcgcaacccctatctttagtagccagcggtatggccgggcactctagagagactgccagggataacctggaggaaggtggggatgacgtcaaatcatcatgccccttatgagcagggctacacacgtgctacaatggcgtaaacaaagggaagcgagcctgcgagggtaagcaaatctcaaaaataacgtctcagttcggattgtagtctgcaactcgactacatgaagctggaatcgctagtaatcgcgaatcagaatgtcgcggtgaatacgttcccgggtcttgtacacaccgcccgtcacaccatgggagttggtaacgcccgaagtcagtgacccaaccgcaaggagggagctgccgaaggtgggaccgataactggggtgaagtcgtaacaaggta

SEQ ID NO: 35 - DNA, 1473 bp, Unknown
  16S rRNA(PAC000195_g)
agagttcgatcctggctcaggataaacgctggcggcgtgcttaacacatgcaagtcgaacgaagtttttctttcgggaggaacttagtggcggacgggtgagtaacgcgtgggtaacctgccctgtacagggggacaacagctggaaacggctgctaataccgcataagcccttagcactgcatggtgcatagggaaaaggagcaatccggtacaggatggacccgcgtctgattagccagttggcagggtaacggcctaccaaagcgacgatcagtagccgatctgagaggatgtacggccacattgggactgagacacggcccagactcctacgggaggcagcagtggggaatattgcacaatggaggaaactctgatgcagcgacgccgcgtgagtgaagaagtatttcggtatgtaaagctctatcagcagggaagaaaatgacggtacctgactaagaagcaccggctaaatacgtgccagcagccgcggtaatacgtatggtgcaagcgttatccggatttactgggtgtaaagggagcgtaggtggcaaggcaagccagaagtgaaaacccggggctcaaccgcgggattgcttttggaactgtcatgctagagtgcaggaggggtgagcggaattcctagtgtagcggtgaaatgcgtagatattaggaggaacaccggaggcgaaggcggctcactggactgtaactgacactgaggctcgaaagcgtggggagcaaacaggattagataccctggtagtccacgcggtaaacgatgaatactagatgtcgggtagcaaagctactcggtgtcgtcgcaaacgcaataagtattccacctggggagtacgttcgcaagaatgaaactcaaaggaattgacggggacccgcacaagcggtggagcatgtggtttaattcgaagcaacgcgaagaaccttacctgctcttgacatcccattcgatagagggtaatgcctctagcccttcgggggaatggagacaggtggtgcatggttgtcgtcagctcgtgtcgtgagatgttgggttaagtcccgcaacgagcgcaacccttattgtcagtagccagcaggtgaagctgggcactctgatgagactgccggggataacccggaggaaggtggggatgacgtcaaatcatcatgccccttatgagcagggctacacacgtgctacaatggcgtaaacagagggaagcgaaggagtgatctggagcaaatctcaaaaataacgtctcagttcggattgtagtctgcaactcgactacatgaagctggaatcgctagtaatcgcagatcagaatgctgcggtgaatacgttcccgggtcttgtacacaccgcccgtcacaccatgggagtcggtaatgcccgaagtcagtgactcaaccgaaaggagagagctgccgaaggcaggactggtaactggggtgaagtcgtaacaaggta

SEQ ID NO: 36 - DNA, 1454 bp, Unknown
  16S rRNA(PAC000196_g)
gatgaacgctggcggcgtgcttaacacatgcaagtcgagcgaagcacttatgatgattcttcggatgaatcatttgtgactgagcggcggacgggtgagtaacgcgtgagtaacctgcctcatacaggggaataacagttagaaatgactgctaatgccgcataagcgcacagggccgcatggcccggtgtgaaaaactccggtggtatgagatggactcgcgtctgattagctagttggcagggtaacggcctaccaaggcgacgatcagtagccggcctgagagggtgaacggccacattgggactgagacacggcccaaactcctacgggaggcagcagtggggaatattgcacaatgggggaaaccctgatgcagcgacgccgcgtgagtgaagaagtatttcggtatgtaaagctctatcagcagggaagaaaatgacggtacctgactaagaagccccggctaactacgtgccagcagccgcggtaatacgtagggggcaagcgttatccggatttactgggtgtaaagggagcgtagacggctttgcaagtctgacgtgaaactccggggctcaactccggaactgcgttggaaactgtaaggcttgagtgccggagaggtaagcggaattcctagtgtagcggtgaaatgcgtagatattaggaggaacaccagtggcgaaggcggcttactggacggcaactgacgttgaggctcgaaagcgtggggagcaaacaggattagataccctggtagtccacgcggtaaacgatgaatactaggtgttgggggacaaagtccttcggtgccgccgcaaacgcattaagtattccacctggggagtacgttcgcaagaatgaaactcaaaggaattgacggggacccgcacaagcggtggagcatgtggtttaattcgaagcaacgcgaagaaccttaccaagtcttgacatcgattcgacgggagtgtaatgactcctttcccttcggggacgaagaagacaggtggtgcatggttgtcgtcagctcgtgtcgtgagatgttgggttaagtcccgcaacgagcgcaacccttatcttcagtagccagcgagtaaggtcggtcactctggagagactgccagggacaacctggaggaaggtggggatgacgtcaaatcatcatgccccttatgacttgggctacacacgtgctacaatggcgtaaacaaagggaagcgaacctgtgagggtgggcaaatcccaaaaataacgtctcagttcggattgtagtctgcaactcgactacatgaagctggaatcgctagtaatcgcgaatcagcatgtcgcggtgaatacgttcccgggtcttgtacacaccgcccgtcacaccatgggagtcggtaacgcccgaagtcagtgacccaaccgcaaggagggagctgccgaaggcgggactggtaactggggtg

SEQ ID NO: 37 - DNA, 1493 bp, Unknown
  16S rRNA(PAC000197_g)
gatgaacgctggcggcatgcctaagacatgcaagtcgtacgaaggggcccaatgaaaagaattgaaattcagagtgcttgcacaaagaatggattttcttggatttggattttccccttagtggcaaacgggtgagtaacacgtgggttacctacctctaagatggggataacagttggaaacgactgataataccgaatgtgctctacggagtaaagaagcccttaaagcttcgcttagagatgggcctgcggcgtattagctagttggtggggcaatggcctaccaaggcgacgatgcgtagccgaactgagaggttgatcggccacactgggactgagacacggcccagactcctacgggagacagcagttaggaatattcgtcaatggaggaaactctgaacgagcaatgccgcgtgaacgatgacggccctatgggttgtaaagttctgttgtttggaaagaacgatagatagaggaaatgctatctatgtgacggtaccattcaagaaagccacggctaactacgtgccagcagccgcggtaatacgtaggtggcgagcgttatccggatttattgggcgtaaagggtgcgcagacggtttattaagtctaaaatcaaatcttggggctcaaccccattccgttttagaaactggtagacttgagtatggtagaggcaaatggaattcctagtgtagcggtggaatgcgtagatattaggaggaacaccagtggcgaaggcgatttgctgggccattactgacgttcaggcacgaaagcgtggggagcaaataggattagataccctagtagtccacgccgtaaacgatgagtactaagtgtcgggttaccggtgctgaagttaacacattaagtactccgcctgagtagtacggtcgcaaggctgaaactcaaaggaattgacgggcacccgcacaagcggtggagcatgctgtttaattcgaaaatacgcgaagaaccttacctaggtttgacatccccggcaaagctatagaaatatagtggaggttatccgggtgacaggtggtgcatggttgtcgtcagctcgtgtcgtgagatgtttggttaagtccaacaacgagcgcaaccctcatcattagttgctaacatttagttgagaactctaatgatactgccagtgtaagctggaggaaggtggggatgaggtcaaatcatcatgccccttacatctagggctacaggcgtgctacaatggccggtacaacgagttgcaacacggtgacgtgaagctaatctcttaaagccggtcccagtccggattggagtctgcaattcgactccatgaagttggaatcgctagtaatcccgaatcagaatgtcggggtgaatacgttcccgggtgttgtacacaccgcccgtcacgccatgggagtctgtaatacttgaagtcggtagcctaacccgtaagggagggggccgcccagggtaggacaggtgactggggtg

SEQ ID NO: 38 - DNA, 1472 bp, Unknown
  16S rRNA(PAC000661_g)
gataaacgctggcggcgcacataagacatgcaagtcgaacggaagtcgttataaaaaggattgaagatttatctgattgagattttataacaatggctttagtggcggactggtgagtaacgcgtgagcaacctgcctactagaggggaataacagtgagaaatcattgctaataccgcatatgccatgaacatcacatgatgaaaatgggaaaagagtaatctgctagtagatgggctcgcgtctgattagatagttggtggggtaacggcctaccaagtcaacgatcagtagccggactgagaggttgaacggccacattgggactgagatacggcccagactcctacgggaggcagcagtcgggaatattgcgcaatggaggaaactctgacgcagtgacgccgcgtataggaagaaggttttcggattgtaaactattgtcgttagggaagatacaagacagtacctaaggaggaagctccggctaactacgtgccagcagccgcggtaatacgtagggagcaagcgttatccggatttattgggtgtaaagggtgcgtagacgggacaacaagttagttgtgaaatccctcggcttaactgaggaactgcaactaaaactattgttcttgagtgttggagaggaaagtggaattcctagtgtagcggtgaaatgcgtagatattaggaggaacaccggtggcgaaggcgactttctggacaataactgacgttgaggcacgaaagtgtggggagcaaacaggattagataccctggtagtccacaccgtaaacgatggatactaggtgtaggaaatgatttcattttctgtgccgtcgcaaacgcaataagtatcccacctggggagtacggccgcaaggttgaaactcaaaggaattgacgggggcccgcacaagcagtggagtatgtggtttaattcgaagcaacgcgaagaaccttaccagggcttgacatatagatgaataactaagagattagttagtccttcgggacatctatacaggtggtgcatggttgtcgtcagctcgtgtcgtgagatgttaggttaagtcctgcaacgagcgcaacccctgtgattagttgccaacaggttaagctgggaactctaatcagactgccggtgataaatcggaggaaggtggggatgacgtcaaatcatcatgccctttatgtcctgggctacacacgtactacaatggctgtaacagagagaagcaacaccgcgaggtagagcgaaactccaaaagcagtctcagttcggattgaaggctgaaattcgccttcatgaagccggaattgctagtaatggcaggtcagcatactgccgtgaatacgttcccgggccttgtacacaccgcccgtcacaccatgagagttgggaatacccgaagcctgtgagccaactgtaaagaggcagcagtcgaaggtagaatcaatgattagggtg

SEQ ID NO: 39 - DNA, 1489 bp, Unknown
  16S rRNA(PAC000692_g)
agagtttgatcctggctcaggatgaacgctggcggcgtgcttaacacatgcaagtcgaacgaagcacttaagattgattcttcggatgacgtcttttgtgacttagtggcggacgggtgagtaacgcgtgggtaacctgcctcacacagggggataacagttagaaatgactgctaataccgcataacccgataggatcgcatgatccagacggaaaagatttatcggtgtgagatggacccgcgtctgattagctagttggtgaggtaacggcccaccaaggcgacgatcagtagccggcctgagagggtgaacggccacattgggactgagacacggcccaaactcctacgggaggcagcagtggggaatattgcacaatgggggaaaccctgatgcagcgacgccgcgtgagtgaagaagtatttcggtatgtaaagctctatcagcagggaagaaaatgacggtacctgactaagaagccccggctaactacgtgccagcagccgcggtaatacgtagggggcaagcgttatccggatttactgggtgtaaagggagcgtagacggtcaagcaagtcagaagtgaaaggctggggctcaaccccgggactgcttttgaaactgtttgactggagtgctggagaggtaagcggaattcctagtgtagcggtgaaatgcgtagatattaggaggaacaccagtggcgaaggcggcttactggacagtaactgacgttgaggctcgaaagcgtggggagcaaacaggattagataccctggtagtccacgccgtaaacgatgaatactaggtgtcggggagcacagctcttcggtgccgccgcaaacgcaataagtattccacctggggagtacgttcgcaagaatgaaactcaaaggaattgacggggacccgcacaagcggtggagcatgtggtttaattcgaagcaacgcgaagaaccttaccaaatcttgacatcccgatgaccgttccgtaatggggacttcccttcggggcatcggtgacaggtggtgcatggttgtcgtcagctcgtgtcgtgagatgttgggttaagtcccgcaacgagcgcaacccttaccttcagtagccagcagttcggctgggcactctggagggactgccagggataacctggaggaaggtggggatgacgtcaaatcatcatgccccttatgatttgggctacacacgtgctacaatggcgtaaacaaagggaagcgagcctgcgagggtaagcaaatctcaaaaataacgtctcagttcggattgtagtctgcaactcgactacatgaagctggaatcgctagtaatcgcgaatcagaatgtcgcggtgaatacgttcccgggtcttgtacacaccgcccgtcacaccatgggagttggtaacgcccgaagtcagtgacctaaccgtaaggaaggagctgccgaaggcgggactgataactggggtgaagtcgtaacaaggta

SEQ ID NO: 40 - DNA, 1449 bp, Unknown
  16S rRNA(PAC000748_g)
gatgaacgctggcggcgtgcttaacacattcaagtcgaacgggactcatttgattaatccttcgggaagcgttgaatgagtttagtggcggacgggtgagtaacgcgtgagcaatttacctttgtgagtggaataacacccggaaacaggtgctaataccgcataacgtatcgatgtcgcatggcaatgataccaaagagaaatcgcacaaagatgagctcgcgtccgattagatagttggtgaggtaacggcccaccaagtcgacgatcggtagccggactgagaggttgaacggccacattggaactgagaaacggtccagactcctacgggaggcagcagtggggaatattgggcaatgggcgaaagcctgacccagcgacgccgcgtgagggaagaaggtcttcggattgtaaaccttagttagcagggaagaagaaagtgacggtacctgcagagaaagccacggctaactacgtgccagcagccgcggtaatacgtaggtggcgagcgttatccggaattactgggtgtaaagggtgtgtaggcgggcagacaagtcagatgtgaaaactatgggcttaacccatagcctgcatttgaaactgtatgtcttgaggatgggagaggtaaatggaattcccggtgtagcggtgaaatgcgtagatatcgggaggaacaccagtggcgaaggcggtttactggaccattactgacgctgagacacgaaagcgtggggagcaaacaggattagataccctggtagtccacgctgtaaacgatgaacactaggtgtaggggagcaatcctctgtgccgcagttaacacaataagtgttccacctggggagtacggccgcaaggttgaaactcaaaggaattgacgggagcccgcacaagcagtggagtatgtggtttaattcgatgcaacgcgaagaaccttaccaggacttgacatcccaagaagaccgatgtaatgttggttgtgcccttcggggaacttggtgacaggtggtgcatggttgtcgtcagctcgtgtcgtgagatgttgggttaagtcccgcaacgagcgcaacccttacggttagttgctacgcaagagcactctaatcggactgccgttgacaaaacggaggaaggtggggatgacgtcaaatcatcatgccccttacgttctgggctacacacgtactacaatggcgaaaacaaagggaagcgaggccgcgaggcggagcaaaccccataaaagtcgtcccagttcagattgtaggctgcaacccgcctgcatgaagtcggaattgctagtaatcgcggatcagcatgccgcggtgaatacgttcccgggctttgtacacaccgcccgtcaaaccatgaaagtcgaaaacacccgaagcctgtgagccaaccgaaagggagcagcagtcgaaggtgggttcggtgattggggtt

SEQ ID NO: 41 - DNA, 1483 bp, Unknown
  16S rRNA(PAC001057_g)
gatgaacgctggcggcatgcctaagacatgcaagtcgaacgagatggcccagtgaaggttgagtgcttgcacaagactgaatctggattcccatctagtggcagacgggtgagtaacacgtgggtgacctaccttttcgttggggataacagttggaaacgattgctaataccgaataaaatgtaagagtcaattttacattgaaaggagcctttaaagcttcgcgattagatgggcctgcggcgtattaactagttggtgaggtaatggcttaccaaggtgacgatgcgtagccgaactgagaggttgatcggccacattgggactgagacacggcccaaactcctacgggagacagcagttaggaatattcgtcaatggaggaaactctgaacgagcaatgccgcgtgagtgatgaaggtcttatagattgtaaaactctgttgtatggaaaaaacgactaggttaggaaatgaacttagtgtgatggtaccataccagaaagccccggctaactacgtgccagcagccgcggtaatacgtagggggcgagcgttatccggatttattgggcgtaaagcgtgtgtaggcggtttattaagtttaagattaaagcccggggctcaactccggtaagtcttaaaaactggtagacttgagtacggtagaggcaaacggaatttctagtgtagcggtgaaatgcgtagatattagaaggaacaccagtggcgaaagcggtttgctgggccgttactgacgctgaggcacgaaagcgtggggagcaaataggattagataccctagtagtccacgccgtaaacgatgagtactaagtgttggggttacccagtgctgaagctaacgtattaagtactccgcctgagtagtacggtcgcaaggctgaaactcaaaggaattgacgggcacccgcacaagcggtggagcatgctgtttaattcgacgatacgcgaagaaccttacctagacttgacatccctggcaaagctatagaaatatagtggaggtcatccaggtgacaggtggtgcatggttgtcgtcagctcgtgtcgtgagatgttcggttaagtccgctaacgagcgcaacccttatccttagttgctaacattaagttgagaaccctaaggagactgccggtgacaaaccggaggaaggtggggatgacgtcaaatcatcatgccccttacgtctagggctacaggcgtgctataatggccgatacaataagaagcaatactgtgaagtggagcaaatctgtaaagtcggtctcagttcggattgaagtctgcaactcgacttcatgaagctagaatcgctagtaatcccaaatcagaatgttggggtgaatacgttcccgggtgttgtacacaccgcccgtcatgccatgaaagtttgtaatacccgaatgtggtagcctaaccttttaggagggggccatttaaggtaggacaagtgattggggta

SEQ ID NO: 42 - DNA, 1439 bp, Unknown
  16S rRNA(PAC001100_g)
gacgaacgctggcggcgtgcctaacacatgcaagtcgaacggagttgaaaggagcttgcttttttcaactcagtggcggacgggtgagtaacgcgtgagtaacctgcctttcagagggggataacgttctgaaaagaacgctaataccgcataagattgtagtttcgcatggagcagcaatcaaaggagcaatccgctgaaagatggactcgcgtccgattagatagttggcggggtaacggcccaccaagtcgacgatcggtagccggactgagaggttgatcggccacattgggactgagacacggcccagactcctacgggaggcagcagtgagggatattgggcaatgggggaaaccctgacccagcaacgccgcgtgagggatgacggttttcggattgtaaacctctgtcctctgtgaagatagtgacggtagcagaggaggaagctccggctaactacgtgccagcagccgcggtaatacgtagggagcaagcgttgtccggatttactgggtgtaaagggtgcgtaggcggattggcaagtcagaagtgaaatccatgggcttaacccatgaactgcttttgaaactgttagtcttgagtgaagtagaggtaggcggaattcccggtgtagcggtgaaatgcgtagagatcgggaggaacaccagtggcgaaggcggcctactgggctttaactgacgctgaggcacgaaagtgtgggtagcaaacaggattagataccctggtagtccacactgtaaacgatgattactaggtgtggggggtctaaccccctccgtgccggagttaacacaataagtaatccacctggggagtacgaccgcaaggttgaaactcaaaggaattgacgggggcccgcacaagcagtggagtatgtggtttaattcgacgcaacgcgaagaaccttaccaggtcttgacatccaactaacgaagcagagatgcgttaggtgcccttcggggaaagttgagacaggtggtgcatggttgtcgtcagctcgtgtcgtgagatgttgggttaagtcccgcaacgagcgcaacccttgtgattagttgctacgcaagagcactctaatcagactgccgttgacaaaacggaggaaggtggggacgacgtcaaatcatcatgccctttatgacctgggctacacacgtactacaatggtcgttaacagagggaagcaataccgcgaggtggagcaaaaccctaaaaacggtctcagttcagattgtaggctgcaactcgcctacatgaagttggaattgctagtaatcgcggatcagcatgccgcggtgaatacgttcccgggccttgtacacaccgcccgtcacaccatgggagccggtaatacccgaagtcagtagtttaaccgtaaggagaacgctgccgaaggtaggattggcgactggggtg

SEQ ID NO: 43 - DNA, 1497 bp, Unknown
  16S rRNA(PAC001109_g)
gatgaacgctggcggcatgcctaagacatgcaagtcgtacgaagtggcccattgatgattgagtgcttgcacaagatttgatttggattcccacttagtggcgcaagggtgagtaacgcgtaggttatctgccttcgagtttggaataacaattagaaatgattgctaatgccggattatatttaagatgatacgttgtcttaaattaaaaggagcctttaaagcttcgcttgaagatgagcctgcgtcgtattagctagttggtggggtaatggcctaccaaggcaacgatgcgtagccgacctgagagggtgatcggccacactgggactgagacacggcccagactcctacgggagacagcagttaggaatattcgtcaatgggggaaaccctgaacgagcaatgccgcgtgaaggatgacggtcctttggattgtaaacttctgttgttagggaagaacaaactgtataggaaatgatacagttctgacggtacctttcaagaaagctccggctaactacgtgccagcagccgcggtaatacgtagggagcaagcgttatccggatttattgggtgtaaagggtgcgtaggcggtttattaggtctatggtttaattccgaagcttaacttcggttcgccatagaaaccgatttacttgagtatggtagaggcaagtggaatttctagtgtagcggtaaaatgcgtagatattagaaggaacaccagtggcgaaggcgacttgctgggccatcactgacgctgaggcacgaaagcgtggggagcaaataggattagataccctagtagtccacgccgtaaacgttgaatactaagtgtcggaatttccggtgctgaagttaacacattaagtattccacctgagtagtacggtcgcaaggctgaaactcaaaggaattgacgggcacccgcacaagcggtggagcatgctgtttaattcgaagatacgcgaagaaccttacctgggcttgacatcccaatgaaagtttttggaaacattaacccttcccttcggggaacattggtgacaggtggtgcatggttgtcgtcagctcgtgtcgtgagatgttcggttaagtccgataacgagcgcaacccttatccttaattgctaacattcagttgagaaccttaaggatactgccggtgacaaaccggaggaaggtggggatgacgtcaaatcatcatgccccttacgtccagggctacaggcgtgctacaatggctggtataataagatgcaatatcgtgagatggagcaaatctctaaagccagtcccagtccggattggagtctgcaactcgactccatgaagttggaatcgctagtaatcccgaatcagaatgtcggggtgaatacgttcccgggtgttgtacacaccgcccgtcacgccatgggagtcgataatacccgaagctggtagcctaaccttttaggagggggccatctaaggtaggatcggtgactggggtg

SEQ ID NO: 44 - DNA, 1440 bp, Unknown
  16S rRNA(PAC001115_g)
gacgaacgctggcggcgtgcttaatacatgcaagtcgaacggagttaagggtttcggcctttaacttagtggcgaacgggtgagtaacgcgtgaataacctgactcaaagagggggataacaacgggaaactgttgctaataccgcatgagaccacaacaccgcatgatgaaggggtcaaagatttatcgctttgagaggggttcgcgtcccattaggtagttggaggggtaacggcccaccaagccaacgatgggtagccgagctgagaggctgatcggccacactggaactgagacacggtccagactcctacgggaggcagcagtagggaatattgggcaatgggcgcaagcctgacccagcaacgccgcgtgagggaagaaggttttcggattgtaaacctctgtcctatgtgacgaaggaagtgacggtagcataggaggaagccccggctaactacgtgccagcagccgcggtaatacgtagggggcgagcgttgtccggaattactgggcgtaaagggtgcgtaggcggtttggtaagttggatgtgaaatacccgggcttaacttgggggctgcatccaatactgtcggacttgagtgcaggagaggaaagcggaattcctagtgtagcggtgaaatgcgtagatattaggaggaacaccggtggcgaaggcggctttctggactgtaactgacgctgaggcacgaaagcgtggggagcaaacaggattagataccctggtagtccacgccgtaaacgatgaatactaggtgtagggggtatagactccctctgtgccgcagcaaacgcaataagtattccgcctggggagtacggccgcaaggttgaaactcaaaggaattgacgggggcccgcacaagcagcggagcatgtggtttaattcgacgcaacgcgaaaaaccttaccaagacttgacatcctactaaactcatggaaacatgaggtgacttcggtcgagtagagacaggtggtgcatggttgtcgtcagctcgtgtcgtgagatgttgggttaagtcccgcaacgagcgcaacccctgttgccggttaccagcgagtaaagtcggggactccggtgagactgccgaggacaactcggaggaaggtggggacgacgtcaaatcatcatgccccttacgtcttgggctacacacgtgctacaatggctgtaacaaagggaagcgacagcgtaagctgaagcggatctcgaaaaggcagtcccagttcggattgtgggctgcaacccgcccacatgaagtcggagttgctagtaatcgcggatcagcatgccgcggtgaatacgttcccgggccttgtacacaccgcccgtcacaccatgggagttgggagcgcccgaagccaatagcctaaccgcaaggagggcgttgtctaaggtgagaccaatgactggggtg

SEQ ID NO: 45 - DNA, 1456 bp, Unknown
  16S rRNA(PAC001137_g)
gatgaacgctggcggcgtgcttaacacatgcaagtcgaacgaagcactttattacgatttcttcggaatgacgatttagtgactgagtggcggacgggtgagtaacgcgtgggtaacctgcctcatacagggggataacagttggaaacgactgctaataccgcataagcgcacggtatcgcatgatacagtgtgaaaaactccggtggtatgagatggacccgcgtctgattagctagttggcgaggtaacggcccaccaaggcaacgatcagtagccgacctgagagggtgaccggccacattgggactgagacacggcccaaactcctacgggaggcagcagtggggaatattgcacaatgggcgaaagcctgatgcagcgacgccgcgtgaacgaagaagtatttcggtatgtaaagttctatcagcagggaagaagaaatgacggtacctgactaagaagctccggctaaatacgtgccagcagccgcggtaatacgtatggagcaagcgttatccggatttactgggtgtaaagggagcgtaggcggtcttataagtctgatgtgaaagcccggggctcaaccccgggactgcattggaaactgtaggactagagtgtcggaggggtaagtggaattcctagtgtagcggtgaaatgcgtagatattaggaggaacaccagtggcgaaggcggcttactggacgattactgacgctgaggctcgaaagcgtggggagcaaacaggattagataccctggtagtccacgccgtaaacgatgaatactaggtgtcggccaccacaggtggtcggtgccgcagcaaacgcaataagtattccacctggggagtacgttcgcaagaatgaaactcaaaggaattgacggggacccgcacaagcggtggagcatgtggtttaattcgaagcaacgcgaagaaccttaccaagtcttgacatccttctgacaaagtatgtaatgtactcttccttcgggacagaagtgacaggtggtgcatggttgtcgtcagctcgtgtcgtgagatgttgggttaagtcccgcaacgagcgcaacccttgtccttagtagccagcatttaaggtgggcactctagggagactgccagggtgaacctggaggaaggtggggatgacgtcaaatcatcatgccccttatgacttgggctacacacgtgctacaatggcgtaaacaaagggaagcgaaatcgcgaggtggagcaaatctcaaaaataacgtctcagttcggattgtagtctgcaactcgactacatgaagctggaatcgctagtaatcgcgaatcagaatgtcgcggtgaatacgttcccgggtcttgtacacaccgcccgtcacaccatgggagttgggaatgcccgaagtcagtgacctaaccgtaaggaaggagctgccgaaggcaggctcgataactggggtg

SEQ ID NO: 46 - DNA, 1445 bp, Unknown
  16S rRNA(PAC001144_g)
gacgaacgctggcggcatgcctaacacatgcaagtcgaacggagatatttggaagcttgcttttggatatcttagtggcggacgggcgagtaacgcgtgagcaacctggccttcagagtggaacaacgtctggaaacgggcgctaataccgcataacacaagagagtcgcatggcttttttgtcaaaggagaaatccgctgaaggatgggctcgcgtccgattagctagatggggtggtaacggcactccatggcgacgatcggtagccgaactgagaggttgatcggccgcattgggactgagacacggcccagactcctacgggaggcagcagtgggggatattggtcaatgggggaaaccctgaaccagcaatgccgcgtgagggaagaaggtcttcggattgtaaacctaagtagtcagggacgaaagaaatgacggtacctgaagagtaagctccggctaactacgtgccagcagccgcggtaatacgtagggagcgagcgttgtccggatttactgggtgtaaagggtgcgtaggcgggatggcaagtcagatgtgaaataccggggcttaaccccggggctgcatttgaaactgtcgttcttgagtgaagtagaggcaggcggaattcctagtgtagcggtgaaatgcgtagatattaggaggaacaccagtggcgaaggcggcctgctgggctttaactgacgctgaggcacgaaagcatggggagcaaacaggattagataccctggtagtccatgccgtaaacgatgattgctaggtgtggggggactgaccccctccgtgccggagtaaacacaataagcaatccacctggggagtacgaccgcaaggttgaaactcaaaggaattgacgggggcccgcacaagcagtggagtatgtggtttaattcgacgcaacgcgaagaaccttaccaggtcttgacatccaactaacgaggtagagatacgtcaggtgcccttcggggaaagttgagacaggtggtgcatggttgtcgtcagctcgtgtcgtgagatgttgggttaagtcccgcaacgagcgcaacccttgtgattagttgctacgcaagagcactctaatcagactgccgttgacaaaacggaggaaggtggggacgacgtcaaatcatcatgccccttatgacctgggctacacacgtactacaatggccgttaacaaagggaagcaaagccgcgaggcggagcaaaaccccaaaaacggtcccagttcagattgcaggctgcaactcgcctgtatgaagttggaattgctagtaatcgcggatcagcatgccgcggtgaatacgttcccgggccttgtacacaccgcccgtcacaccatgggagccggtaatacccgaagtcagtagcctaaccgcaaggagggcgctgccgaaggtaggattggcgactggggtga

SEQ ID NO: 47 - DNA, 1437 bp, Unknown
  16S rRNA(PAC001168_g)
gatgaacgctggcggcgtgcctaacacatgcaagtcgagcgagaagctcgtgacagacgcttcggttgaagtcacgagtggaaagcggcggacgggtgagtaacgcgtaggcaacctgccctttgcagagggatagcctcgggaaaccgggattaaaacctcataataccgcagtgagacatctcacagtggtcaaagatttatcggcaaaggatgggcctgcgtctgattagttagttggtggggtaacggcctaccaaggcgacgatcagtagccgacctgagagggtgatcggccacattggaactgagacacggtccaaactcctacgggaggcagcagtggggaatattgcacaatgggggaaaccctgatgcagcaacgccgcgtgaaggatgaaggcctttgggtcgtaaacttctgttctaagggaagatagtgacggtaccttaggagcaagtcccggctaactacgtgccagcagccgcggtaatacgtagggggcaagcgttatccggaattattgggcgtaaagagtacgtaggtggttttctaagcacggggtttagggcaatggcttaaccattgttcgccttgtgaactggaagacttgagtgcaggagaggaaagcggaattcctagtgtagcggtgaaatgcgtagatattaggaggaacaccagtggcgaaggcggctttctggactgtaactgacactgaggtacgaaagcgtggggagcgaacaggattagataccctggtagtccacgccgtaaacgatgagcactaggtgtcgggggtcgcaagacttcggtgccgcagttaacgcattaagtgctccgcctggggagtacgttcgcaagaatgaaactcaaaggaattgacggggacccgcacaagcagcggagcatgtggtttaattcgaagcaacgcgaagaaccttaccagggcttgacatccctctgacagatccttaaacggatccttcttcggacagaggagacaggtggtgcatggttgtcgtcagctcgtgtcgtgagatgttgggttaagtcccgcaacgagcgcaacccttgtcattagttgccagcagtaagatgggcactctagtgagactgccggggataactcggaggaaggtggggatgacgtcaaatcatcatgccccttatgttctgggctacacacgtgctacaatggccggtacagagagaagccagaccgcgaggtggagcaaaactcaaaagccggtcccagttcggattgcaggctgcaactcgcctgcatgaagtcggagttgctagtaatcgcagatcagaatgctgcggtgaatgcgttcccgggtcttgtacacaccgcccgtcacaccatggaagttgggggcgcccgaagttggtcgagaaatagattacctaaggcgaaatcaatgactggggtg

SEQ ID NO: 48 - DNA, 1440 bp, Unknown
  16S rRNA(PAC001177_g)
agagtttgatcctggctcaggatgaacgctggcggcgtgcttaacacatgcaagtcgaacgaagcactttggacagattcttcggatgaagtccttagtgactgagtggcggacgggtgagtaacgcgtgggtaacctgcctcatacagggggataacagttagaaatggctgctaataccgcataagcgcacggtactgcatggtacagtgtgaaaaactccggtggtatgagatggacccgcgttggattagctagttggcagggtaacggcctaccaaggcgacgatccatagccggcctgagagggtggacggccacattgggactgagacacggcccagactcctacgggaggcagcagtggggaatattgcacaatgggggaaaccctgatgcagcgacgccgcgtgagcgaagaagtatttcggtatgtaaagctctatcagcagggaagaaaatgacggtacctgactaagaagccccggctaactacgtgccagcagccgcggtaatacgtagggggcaagcgttatccggatttactgggtgtaaagggagcgtagacggaatggcaagtctgatgtgaaaggccggggctcaaccccgggactgcattggaaactgtcaatctagagtaccggaggggtaagtggaattcctagtgtagcggtgaaatgcgtagatattaggaggaacaccagtggcgaaggcggcttactggacggtaactgacgttgaggctcgaaagcgtggggagcaaacaggattagataccctggtagtccacgccgtaaacgatgaatactaggtgttggggagcaaagctcttcggtgccgcagcaaacgcaataagtattccacctggggagtacgttcgcaagaatgaaactcaaaggaattgacggggacccgcacaagcggtggagcatgtggtttaattcgaagcaacgcgaagaaccttaccaaatcttgacatcgatctgaccggactgtaatgagtcctttcccttcggggacagagaagacaggtggtgcatggttgtcgtcagctcgtgtcgtgagatgttgggttaagtcccgcaacgagcgcaacccttatcctcagtagccagcaagtgaagttgggcactctgtggagactgccagggataacctggaggaaggtggggatgacgtcaaatcatcatgccccttatgatttgggctacacacgtgctacaatggcgtaaacaaagggaagcgatcacgcgagtgtgagcaaatctcaaaaataacgtctcagttcggattgtagtctgcaactcgactacatgaagctggaatcgctagtaatcgcaggtcagcatactgcggtgaatacgttcccgggtcttgtacacaccgcccgtcacaccatgggagtcagtaacacccgaagccggtgacctaaccgaaagg

SEQ ID NO: 49 - DNA, 1486 bp, Unknown
  16S rRNA(PAC001200_g)
agagtttgatcctggctcaggatgaacgctggcggcgtgcttaacacatgcaagtcgaacgaggaattttaaatgagacttcggtggattttgaaattcttagtggcggacgggtgagtaacgcgtgggcaacctgccctgtacagggggacaacagctggaaacggctgctaataccgcataagcgcacagcatcgcatgatgccgtgtgaaaaactccggtggtacaggatgggcccgcgttggattaggtagttggtggggtaacggcctaccaagccgacgatccatagccgacctgagagggtgaccggccacattgggactgagacacggcccaaactcctacgggaggcagcagtggggaatattgcacaatgggggaaaccctgatgcagcgacgccgcgtgagcgaagaagtatttcggtatgtaaagctctatcagcagggaagaaaatgacggtacctgactaagaagccccggctaactacgtgccagcagccgcggtaatacgtagggggcaagcgttatccggatttactgggtgtaaagggagcgtagacggctttgcaagtctgatgtgaaaggcgggggctcaacccctggactgcattggaaactgtgaggcttgagtgccggagaggtaagcggaattcctagtgtagcggtgaaatgcgtagatattaggaggaacaccagtggcgaaggcggcttactggacggtaactgacgttgaggctcgaaagcgtggggagcaaacaggattagataccctggtagtccacgcggtaaacgatgaatactaggtgttgggtgtcacagacattcggtgccgcagcaaacgcaataagtattccacctggggagtacgttcgcaagaatgaaactcaaaggaattgacggggacccgcacaagcggtggagcatgtggtttaattcgaagcaacgcgaagaaccttaccaagtcttgacatctccctgacagagtatgtaatgtacttttccttcgggacagggaagacaggtggtgcatggttgtcgtcagctcgtgtcgtgagatgttgggttaagtcccgcaacgagcgcaacccttatcctcagtagccagcggttcggccgggcactctgtggagactgccagggataacctggaggaaggtggggatgacgtcaaatcatcatgccccttatgacttgggctacacacgtgctacaatggcgtaaacaaagggaagcgagagagcgatctggagcaaatcccaaaaataacgtcccagttcggattgtagtctgcaactcgactacatgaagctggaatcgctagtaatcgcgaatcagaatgtcgcggtgaatacgttcccgggtcttgtacacaccgcccgtcacaccatgggagtcggtaacgcccgaagtcagtgacccaaccgaaaggagggagctgccgaaggcgggactggtaactggggtgaagtcgtaacaaggta

SEQ ID NO: 50 - DNA, 1450 bp, Unknown
  16S rRNA(PAC001201_g)
gatgaacgccggcggcacgcttaacacatgcaagtcgagcggagttttgtgcggaagattcggttggaagtataaaacttagcggcggacgggtgaggaacgcgtgggtaacctgccctgtacagggggataacacggagaaatctgtgctaaaaccgcataagctcacgggaccgcatggtcttgggagaaaaactccggtggtacaggatgggcccgcgtctgattagctagttggagaggtaagagctcaccaaggcgacgatcagtagccggtctgagaggatggacggccacattgggactgagacacggcccaaactcctacgggaggcagcagtggggaatattgcacaatgggggaaaccctgatgcagcgatgccgcgtgaaggaagaagattttcggattgtaaacttctatcagcaaggaagaaaacggacagtacttgagtaagaagccccggctaactacgtgccagcagccgcggtaatacgtagggggcgagcgttatccggaattactgggtgtaaagggtgcgtaggcggtacggcaagtttgatgtgaaacccgcgggcttaacccgaggcatgcatcgaaaactactgaactagagtgcaggagaggaaagcggaattcctagtgtagcggtgaaatgcgtagatattaggaagaacaccagtggcgaaggcggctttctggactgcaactgacgctgaggcacgaaagcgtggggagcaaacaggattagataccctggtagtccacgccgtaaacgatgaatgctaggtgttgggttctgaaggactcggtgccgcagttaacgcaataagcattccacctggggagtacgaccgcaaggttgaaactcaaaggaattgacgggggcccgcacaagcggtggagcatgtggattaattcgacgcaacgcgaagaaccttaccaggtcttgacatccctctgaatactgtagagatatggtaggccttcgggacagaggagacaggtggtgcatggttgtcgtcagctcgtgtcgtgagatgttgggttaagtcccgcaacgagcgcaacccttatcgatagtagccagcaaggaaggttgggcactctattgagactgccggggataactcggaggaaggtggggatgacgtcaaatcatcatgccccttatgacctgggcttcacacgtgctacaatggctgtcacaaagagaagcgagcccgcgagggggagcgaagctcaaaaaggcagtcccagttcggattgcaggctgcaacccgcctgcatgaagctggaatcgctagtaatcgcgaatcagcatgtcgcggtgaatacgttcccgggccttgtacacaccgcccgtcacaccatgggagtttagagcacccgaagtcagtgaggtaaccgaaaggagccagctgccgaaggtgagctaagtaactggggtg

SEQ ID NO: 51 - DNA, 1445 bp, Unknown
  16S rRNA(PAC001207_g)
gacgaacgctggcggcgtgcctaacacatgcaagtcgagcggagacagtgagtagcttgctacgaactgttttagcggcggacgggtgagtaacgcgtgagcaacctttcccagacaggggaataacacaccgaaaggtgtactaataccgcataagaccacgggatcacatggttctggggtaaaagatttatcggtttggggtgggctcgcgtccgattaggtagttggtgaggtaacggcccaccaagccgacgatcggtagccgacctgagagggtgatcggccacattgggactgagacacggcccaaactcctacgggaggcagcagtggggaatattgggcaatggggggaaccctgacccagcaacgccgcgtggaggaagaaggttttcggatcgtaaactcctgtccttggagacgagtagaagacggtatccaaggaggaagccccggctaactacgtgccagcagccgcggtaatacgtagggggcaagcgttgtccggaataattgggcgtaaagggcgcgtaggcggctcggtaagtctggagtgaaagtcctgcttttaaggtgggaattgctttggatactgtcgggcttgagtgcaggagaggttagtggaattcccagtgtagcggtgaaatgcgtagagattgggaggaacaccagtggcgaaggcgactaactggactgtaactgacgctgaggcgcgaaagtgtggggagcaaacaggattagataccctggtagtccacactgtaaacgatgaatgctaggtgtagggggtatcgaccccttctgtgccgcagtcaacacaataagcattccgcctggggagtacggccgcaaggttgaaactcaaaggaattgacgggggcccgcacaagcagcggagcatgtggtttaattcgacgcaacgcgaagaaccttaccaggtcttgacatccacttaaacttacagagatgtaaggtgtgcttgcacaaagtgagacaggtggtgcatggttgtcgtcagctcgtgtcgtgagatgttgggttaagtcccgcaacgagcgcaacccttatcttcagttactaacgcgtagaggtgaggactctgaagagactgccggggacaactcggaggaaggtggggacgacgtcaaatcatcatgccccttatgacctgggctacacacgtgctacaatggccacgacagagagaagcgaaatcgcaaggtagagcggaactcaaaaaagtggtcccagttcggattgtgggctgcaacccgcccacatgaagtcggagttgctagtaatcgcggatcagcatgccgcggtgaatacgttcccgggccttgtacacaccgcccgtcacaccatgggagttgggagtgcccaaagccggtgaggcaaccgcaaggagccagccgtctaaggcaagaccaatgactggggtg

SEQ ID NO: 52 - DNA, 1448 bp, Unknown
  16S rRNA(PAC001217_g)
gacgaacgctggcggcgtgcctaacacatgcaagtcgaacggggttacacgaggtgcttgcaccatgtggaacctagtggcggacgggtgagtaacgcgtgagcaacctgcctttcagagggggataacaacgggaaaccgttgctaataccgcataataccggatgatggcatcattgaccggtcaaaggagcaatccgctgaaagatgggctcgcgtcccattaggtagttggtggggtaaaggcctaccaagccgacgatgggtagccggactgagaggttgatcggccacattggaactgagacacggtccaaactcctacgggaggcagcagtggggaatattgggcaatgggggaaaccctgacccagcaacgccgcgtggaggaagaaggtcttcggattgtaaactcctgtccttagggaagaaacaaatgacggtacctgaggaggaagctccggctaactacgtgccagcagccgcggtaatacgtagggagcgagcgttgtccggaattactgggcgtaaagggtgcgtaggcggtctgaaaagtcggatgtgaaatccccgtgcttaacatgggagctgcattcgaaactttcggacttgagtgtcggagaggtaagcggaattcccggtgtagcggtgaaatgcgtagatatcgggaggaacaccagtggcgaaggcggcttactggacgacaactgacgctgaggcacgaaagcgtggggagcaaacaggattagataccctggtagtccacgccgtaaacgatggatactaggtgtaggaggtaacacccctcctgtgccgcagccaacgcaataagtatcccgcctggggagtacgatcgcaagattgaaactcaaaggaattgacgggggcccgcacaagcagcggagcatgtggtttaattcgaagcaacgcgaagaaccttaccaagacttgacatcccttgacaggcatggaaacatgctttcccttcggggcaaggagacaggtggtgcatggttgtcgtcagctcgtgtcgtgagatgttgggttaagtcccgcaacgagcgcaacccttacacttagttaccagcgggtaaagccggggactctaagtggactgccggggacaactcggaggaaggtggggacgacgtcaaatcatcatgccccttatgtcttgggctacacacgtgctacaatggccgttacaaagagcagcgagagggtaacctggagcgaaactcaaaaaagcggtcccagttcggattgtgggctgcaacccgcccacatgaagtcggagttgctagtaatcgcggatcagcatgccgcggtgaatgcgttcccgggccttgtacacaccgcccgtcacaccatgggagttgggagcacccgaagccggtgacttaaccgcaaggagagagccgtcgaaggtgagatcaataactagggtg

SEQ ID NO: 53 - DNA, 1340 bp, Unknown
  16S rRNA(PAC001219_g)
gacgaacgctggcggcgtgcttaacacatgcaagtcgaacgggcgtagcaatacgtcagtggcggacgggtgagtaacgcgtgagcaatctgcctctgtcagggggataacacttagaaataggtgctaataccgcataagaccacgtttcggcatcggagagtggtgaaagatttatcggacagagatgagctcgcgtcccattagctagttggtaaggtaacggcctaccaaggcgacgatgggtagccgacctgagagggtgatcggccacactggaactgagaaacggtccagactcctacgggaggcagcagtggggaatattgggcaatggagggaactctgacccagcaacgccgcgtgaaggaagaaggttttcggattgtaaacttctgtcgcgagggacgaagaatgacggtacctcgtaagaaagccccggctaactacgtgccagcagccgcggtaatacgtagggggcaagcgttgtccggaatgactgggcgtaaagggagtgtaggcggcttggcaagttagatgtgaaagcccgcagctcaactgcggaactgcatctaaaactgtcaggcttgagtgcaggagaggtaagtggaattcctagtgtagcggtggaatgcgtagatattaggaggaacaccagaggcgaaggcgacttactggactgtaactgacgctgaggctcgaaagcgtggggagcaaacaggattagataccctggtagtccacgccctaaacgatggatactggacgaagcggatataaagtctgctgtgtcgaagcaaacgcgataagtatcccgcctgaggagtacggccgcaaggttgaaactcaaagaaattgacggggacccgcacaagcagcggagcatgtggattaattcgaagcaacgcgaagaaccttaccaagacttgacatcgtacgacagactgtgaaagcagtttttcctttgggacgtatagacaggtggtgcatggttgtcgtcagctcgtgtcgtgagatgttcggttaagtccggcaacgagcgcaacccttatgaacagttgccaatattaagttaggaactctgttcagactgccgtggataacacggaggaaggtggggatgacgtcaaatcatcatgccccttacgtcttgggcctcacacgtgctacaatgggcgtaacaaagagcagcgagaccgtaaggttaagcgaatctcaaaaaagcgttctcagttcggattgtgggctgcaacccgcccacatgaagtcggagttgctagtaatcccgaatcagaatgtcggggtgaatgcgttcccgggtcttgtacacaccgcccgtc

SEQ ID NO: 54 - DNA, 1442 bp, Unknown
  16S rRNA(PAC001231_g)
gatgaacgctggcggcgtgcctaacacatgcaagtcgaacggagtttacatgaaacctagtgattgtaaacttagtggcggacgggtgagtaacgcgtgggtaacctgccctgtactgggggataacacttagaaataggtgctaataccgcataagcgcacagtgccgcatggcacagtgtgaaaaactccggtggtacaggatggacccgcgtctgattagatagttggtgaggtaacggcccaccaagtcaacgatcagtagccggcctgagagggtgaacggccacattgggactgagacacggcccaaactcctacgggaggcagcagtggggaatattgcacaatgggggaaaccctgatgcagcgacgccgcgtgagtgaagaagtatttcggtatgtaaagctctatcagcagggaagaaaatgacggtacctgactaagaagccccggctaactacgtgccagcagccgcggtaatacgtagggggcaagcgttatccggatttactgggtgtaaagggagcgtagacggtgagacaagtctgaagtgaaatcccggggctcaaccccggaactgctttggaaactgcctgactagagtgcaggagaggtaagtggaattcctagtgtagcggtgaaatgcgtagatattaggaggaacaccagtggcgaaggcggcttactggactgtaactgacgttgaggctcgaaagcgtggggagcaaacaggattagataccctggtagtccacgcggtaaacgatgattactaggtgtcgggggtttataaaccttcggtgccgccgcaaacgcaataagtaatccacctggggagtacgttcgcaagaatgaaactcaaaggaattgacggggacccgcacaagcggtggagcatgtggtttaattcgaagcaacgcgaagaaccttacctggtcttgacatcccgatgaataacgtgtaatggcgttagtacttcggtacattggagacaggtggtgcatggttgtcgtcagctcgtgtcgtgagatgttgggttaagtcccgcaacgagcgcaacccttatctttagtagccagcagtaagatgggaactctagagagactgccggggataacccggaggaaggtggggatgacgtcaaatcatcatgccccttatgaccagggctacacacgtgctacaatggcgtaaacaaagggaagcgaaaccgcgaggtggagccaatcccaaaaataacgtcccagttcggattgtagtctgcaactcgactacatgaagctggaatcgctagtaatcgcagatcagaatgctgcggtgaatacgttcccgggtcttgtacacaccgcccgtcacaccatgggagtcggaaatgcccgaagccggtgacctaaccgaaaggaaggagccgtcgaaggcaggtctgataactggggtg

SEQ ID NO: 55 - DNA, 1439 bp, Unknown
  16S rRNA(PAC001236_g)
gatgaacgctggcggcgtgcctaacacatgcaagtcgagcgagaagtcatggatggaatcttcggaggaaagaaatgatggaaagcggcggacgggtgagtaacgcgtaggtaacctgccccatacagagggatagccactggaaacggtgattaatacctcatgacactttctcttcgcatggagaggaggtcaaagatttatcggtatgggatggacctgcgtctgattagcttgttggtggggtaacggcctaccaaggcgacgatcagtagccgacctgagagggtgatcggccacattggaactgagacacggtccaaactcctacgggaggcagcagtggggaatattgcacaatgggggaaaccctgatgcagcaacgccgcgtgaaggaagaaggcctttgggtcgtaaacttctgttctgagggaagaagaaagtgacggtacctcaggagaaagccccggctaactacgtgccagcagccgcggtaatacgtagggggcaagcgttgtccggaattattgggcgtaaagagtacgtaggcggtttgctaagcgcaaggtgaaaggcagtggcttaaccattgtaagccttgcgaactgacagacttgagtgcaggagaggaaagcggaattcctagtgtagcggtgaaatgcgtagatattaggaggaacaccggtggcgaaggcggctttctggactgtaactgacgctgaggtacgaaagcgtggggagcaaacaggattagataccctggtagtccacgccgtaaacgatgagcactaggtgtcgggatcgtaggatttcggtgccgcagttaacgcattaagtgctccgcctggggagtacgcacgcaagtgtgaaactcaaaggaattgacggggacccgcacaagcagcggagcatgtggtttaattcgaagcaacgcgaagaaccttaccaggacttgacatccctctgacagagccttaaccggctccttcttcggacagaggagacaggtggtgcatggttgtcgtcagctcgtgtcgtgagatgttgggttaagtcccgcaacgagcgcaacccttgtcattagttactaacattaagttgaggactctaatgagactgccggggacaactcggaggaaggtggggatgacgtcaaatcatcatgccccttatgttctgggctacacacgtgctacaatggccggtacaaagagaagcaagaccgcgaggtggagcgaaactcaaaaaccggtcccagttcggactgcaggctgcaactcgcctgcacgaagttggagttgctagtaatcgcggatcagaatgccgcggtgaatgcgttcccgggtcttgtacacaccgcccgtcacaccatggaagttgggggcgcccgaagttggtcgagaaatagattacctaaggcgaaaccaatgactggggtg

SEQ ID NO: 56 - DNA, 1448 bp, Unknown
  16S rRNA(PAC001247_g)
gacgaacgctggcggcgcgcctaacacatgcaagtcgaacggagattacaggcggaagttttcggatggaagcttgtaaacttagtggcggacgggtgagtaacacgtgagcaacctgcctatcagagggggataacgattggaaacgatcgctaataccgcatgacatagcggaatcgcatggttctgttatcaaagattttatcgctgatagatgggctcgcgtccgattagatagttggtggggtaacggcctaccaagtcgacgatcggtagccggactgagaggtcgaacggccacattgggactgagacacggcccagactcctacgggaggcagcagtgggggatattgcacaatgggggaaaccctgatgcagcgacgccgcgtgagggaagacggtcctctggattgtaaacctctgtcttcggggacgaaacgagacggtacccgaggaggaagccacggctaactacgtgccagcagccgcggtaatacgtaggtggcaagcgttgtccggaattactgggtgtaaagggagcgtaggcgggcaggcaagtcaggcgtgaaatatatcggctcaaccggtaacggcgcttgaaactgcaggtcttgagtgaagtagaggttggcggaattcctagtgtagcggtgaaatgcgtagatattaggaggaacaccagtggcgaaggcggccaactgggcttttactgacgctgaggctcgaaagtgtggggagcaaacaggattagataccctggtagtccacaccgtaaacgatgattactaggtgtggggggactgaccccttccgtgccggagttaacacaataagtaatccacctggggagtacggccgcaaggttgaaactcaaaggaattgacgggggcccgcacaagcagtggagtatgtggtttaattcgacgcaacgcgaagaaccttaccaggtcttgacatcgtatgcatagtgtagagatacatgaagtccttcgggacatacagacaggtggtgcatggttgtcgtcagctcgtgtcgtgagatgttgggttaagtcccgcaacgagcgcaacccttgtatttagttgctacgcaagagcactctagatagactgccgtggacaacacggaggaaggtggggatgacgtcaaatcatcatgccccttatgacctgggctacacacgtactacaatggcaatagaacagagggaagcgactcagcgatgagaagcagatcccgaaaaattgtctcagttcggattgcaggctgcaacccgcctgcatgaagtcggaattgctagtaatcgcggatcagcatgccgcggtgaatacgttcccgggccttgtacacaccgcccgtcacaccatgggagtcggtaacacccgaagcccgtagcctaacagcaatgagggcgcggtcgaaggtgggattgatgactggggtg

SEQ ID NO: 57 - DNA, 1489 bp, Unknown
  16S rRNA(PAC001274_g)
gatgaacgctggcggcatgcctaagacatgcaagtcgaacgaggtggcccaaagaagattgagtgcttgcacaagattggacttggattaccacctagtggcggacgggtgagtaacacgtaggtgacctgcctttgagtttgggataactattagaaatgatagctaataccgaattaaatgcagattcgtttctgtattaaaaggagcctttaaagcttcgcttaaagatgggcctgcggcgtattagctagttggtgaggtaatggcttaccaaggcgacgatgcgtagccgaactgagaggttgatcggccacattgggactgagacacggcccaaactcctacgggagacagcagttaggaatattcgtcaatgggggaaaccctgaacgagcaatgccgcgtgaacgatgaaggccctatgggttgtaaagttctgttgcatgggacgaacgattaggataggaaatgatcttaatgtgacggtaccatgccagaaagctccggctaactacgtgccagcagccgcggtaatacgtagggagcaagcgttatccggatttattgggcgtaaagggtgcgtaggcggcttgttaagtatgagattaaagcccgaggcttaacctcggttcgtttcataaactggcaggcttgagtgtggcagaggtaaacggaatttctagtgtagcggttaaatgcgtagatattagaaggaacaccagtggcgaaggcggtttactgggccataactgacgctgaggcacgaaagcgtggggagcaaataggattagataccctagtagtccacgccgtaaacgatgagtactaagtgttggggcaacccagtgctgaagttaacacattaagtactccgcctgagtagtacggtcgcaaggctgaaactcaaaggaattgacgggcacccgcacaagcagtggagcatgctgtttaattcgaagatacgcgaagaaccttaccagggcttgacatcccactgaccgctttagaaataaggctttcccttcggggacagtggtgacaggtggtgcatggttgtcgtcagctcgtgtcgtgagatgttcggttaagtccgataacgagcgcaacccttttctctaattgctaacattcagttgagaaccttagagatactgccggtgacaaaccggaggaaggtggggatgacgtcaaatcatcatgccccttacgtcctgggctacaggcgtgctataatggcagatataaaaagtcgcaaaaccgtgaggtggagctaatctgtaaagtctgtctcagttcggattgaagtctgcaactcgacttcatgaagctagaattgctagtaatcgtggatcagaatgccacggtgaatacgttcccgggtgttgtacacaccgcccgtcacgccatgggagtctgtaatatctaaaaatggtagcctaaccgtttacggagggatccatctaaggtaggacaggtgactggggtg

SEQ ID NO: 58 - DNA, 1500 bp, Unknown
  16S rRNA(PAC001283_g)
agagtttgatcctggctcaggatgaacgctggcggcgtgcctaacacatgcaagtcgaacggagatgcgatgtgagcgagaggtgcttgcactgattaatcttttcgtatcttagtggcggacgggtgagtaacgcgtgggtaacctgccttataccgggggataacacttagaaataggtgctaataccgcataagcgcacggtgtcgcatgacacagtgtgaaaaactccggtggtataagatggacccgcgtctgattagccagttggcagggtaacggcctaccaaagcgacgatcagtagccggcctgagagggtgaacggccacattgggactgagacacggcccaaactcctacgggaggcagcagtggggaatattgcacaatgggggaaaccctgatgcagcgacgccgcgtgagtgaagaagtatttcggtatgtaaagctctatcagcagggaagaagaaatgacggtacctgactaagaagccccggctaactacgtgccagcagccgcggtaatacgtagggggcaagcgttatccggatttactgggtgtaaagggagcgtagacggtgaagcaagtctgaagtgaaaggttggggctcaaccccgaaactgctttggaaactgtttaactggagtacaggagaggtaagtggaattcctagtgtagcggtgaaatgcgtagatattaggaggaacaccagtggcgaaggcggcttactggactgtaactgacgttgaggctcgaaagcgtggggagcaaacaggattagataccctggtagtccacgccgtaaacgatgattactaggtgttggtggatatggatccatcggtgccgcagcaaacgcaataagtaatccacctggggagtacgttcgcaagaatgaaactcaaaggaattgacggggacccgcacaagcggtggagcatgtggtttaattcgaagcaacgcgaagaaccttacctgatcttgacatccctatgaatacagggtaatgcctgtagtacttcggtacataggagacaggtggtgcatggttgtcgtcagctcgtgtcgtgagatgttgggttaagtcccgcaacgagcgcaacccctatctttagtagccagcagtaagatgggcactctagagagactgccggggataacccggaggaaggtggggatgacgtcaaatcatcatgccccttatgaccagggctacacacgtgctacaatggcgtaaacagagggaagcgaagtggtgacatggagcaaatcccaaaaataacgtcccagttcggattgcaggctgcaactcgcctgcatgaagctggaatcgctagtaatcgcagatcagaatgctgcggtgaatacgttcccgggtcttgtacacaccgcccgtcacaccatgggagtaggtaatgcccgaagtcggtgacctaaccgcaaggaaggagccgccgaaggcaggacttataactggggtgaagtcgtaacaaggta

SEQ ID NO: 59 - DNA, 1458 bp, Unknown
  16S rRNA(PAC001296_g)
gatgaacgctggcggcgtgcttaacacatgcaagtcgaacgaagcactttactacgattccttcgggatgacggtttggtgactgagtggcggacgggtgagtaacgcgtggggaacctgccccataccgggggataacagccggaaacggctgctaataccgcataagcgcacagtaccgcatggtacggtgtgaaaaactccggtggtatgggatggacccgcgtctgattagccagttggcgggggtaacggcccaccaaagcgacgatcagtagccggcctgagagggcgaccggccacattgggactgagacacggcccagactcctacgggaggcagcagtggggaatattgcacaatgggggaaaccctgatgcagcgacgccgcgtgagtgaggaagtatttcggtatgtaaagctctatcagcagggaagaagaaatgacggtacctgactaagaagccccggctaactacgtgccagcagccgcggtaatacgtagggggcaagcgttatccggatttactgggtgtaaagggagcgcaggcggcatgataagtctgatgtgaaaacccaaggctcaaccatgggactgcattggaaactgtcgtgctggagtgtcggagaggtaagcggaattcctagtgtagcggtgaaatgcgtagatattaggaggaacaccagtggcgaaggcggcttactggacgatgactgacgctgaggctcgaaagcgtggggagcaaacaggattagataccctggtagtccacgccgtaaacgatgaatactaggtgtcggggagcacagctcttcggtgccgcagcaaacgcagtaagtattccacctggggagtacgttcgcaagaatgaaactcaaaggaattgacggggacccgcacaagcggtggagcatgtggtttaattcgaagcaacgcgaagaaccttaccaagtcttgacatccttctgacagagtatgtaatgtactttctcttcggggcagaagtgacaggtggtgcatggttgtcgtcagctcgtgtcgtgagatgttgggttaagtcccgcaacgagcgcaacccttatccttagtagccagcacgcagtggtgggcactctggggagactgccagggataacctggaggaaggtggggatgacgtcaaatcatcatgccccttatgacttgggctacacacgtgctacaatggcgtaaacaaagggaagcgagcccgtgagggggagcaaatcccaaaaataacgtcccagttcggattgtagtctgcaactcgactacatgaagctggaatcgctagtaatcgcgaatcagaatgtcgcggtgaatacgttcccgggtcttgtacacaccgcccgtcacaccatgggagtcgggaatgcccgaagccggtgacctaacctacgggaaggagccgtcgaaggcagattcgataactggggtg

SEQ ID NO: 60 - DNA, 1454 bp, Unknown
  16S rRNA(PAC001398_g)
gatgaacgctggcggcgtgcttaacacatgcaagtcgaacgaagcacttttgctgagaccttcgggtggatttaaaagtgactgagtggcggacgggtgagtaacgcgtgggtaacctgcctcacacagggggataacagttagaaatgtctgctaataccgcataagcgcacggtctcgcatgggacagtgtgaaaaactccggtggtgtgagatggacccgcgtctgattagctagttggtggggtaacggcctaccaaggcgacgatcagtagccgacctgagagggtgaccggccacattgggactgagacacggcccaaactcctacgggaggcagcaagtggggaatattgcacaatgggggaaaccctgatgcagcgacgccgcgtgattgaagaagtatttcggtatgtaaagatctatcagcaaggaagaaaatgacggtacttgactaagaagccccggctaactacgtgccagcagccgcggtaatacgtagggggcaagcgttatccggatttactgggtgtaaagggagcgtaggcggtctggcaagccagaagtgaaagcccggggcttaaccccgggactgcttttggaactgttagactagagtgtcggagaggtaagtggaattcctagtgtagcggtgaaatgcgtagatattaggaggaacaccagtggcgaaggcggcttactggacgataactgacgctgaggctcgaaagcgtggggagcaaacaggattagataccctggtagtccacgccgtaaacgatgaatactaggtgttggggagcatggctcttcggtgccgcagcaaacgcaataagtattccacctggggagtacgttcgcaagaatgaaactcaaaggaattgacggggacccgcacaagcggtggagcatgtggtttaattcgaagcaacgcgaagaaccttaccaagtcttgacatcccgatgaccgttccgtaatggggacttctcttcgcagcatcggtgacaggtggtgcatggttgtcgtcagctcgtgtcgtgagatgttgggttaagtcccgcaacgagcgcaacccctatcttcagtagccagcattttggatgggcactctggagagactgccagggataacctggaggaaggtggggatgacgtcaaatcatcatgccccttatgacttgggctacacacgtgctacaatggcgtaaacaaagagaagcgaagctgtgaggcagagcaaatctcaaaaataacgtctcagttcggattgtagtctgcaactcgactacatgaagctggaatcgctagtaatcgcgaatcagaatgtcgcggtgaatacgttcccgggtcttgtacacaccgcccgtcacaccatgggagtcagtaacgcccgaagtcagtgacctaaccgcaaggaaggagctgccgaaggcgggaccgataactggggtg

SEQ ID NO: 61 - DNA, 1449 bp, Unknown
  16S rRNA(PAC001435_g)
gacgaacgctggcggcgtgcttaacacatgcaagtcgaacgaaccgtagaaatacggttagtggcggacgggtgagtaacgcgtgagcaatctgcccttgtcaggggaataacacaaagaaatttgtgctaataccgcataatatcagagaacggcatcgttcactgatcaaagaattatcggacaaggatgagctcgcgtcccattaggtagttggtgaggtaacggcccaccaagccgacgatgggtagccgacctgagggggtgatcggccacattggaactgagaaacggtccagactcctacgggaggcagcagtggggaatattgggcaatggaggcaactctgacccagcaacgccgcgtgaatgatgaaggtcttcggattgtaaagttctgtgacgggggacgaagaaagtgacggtaccccgatagcaagctacggctaactacgtgccagcagccgcggtaatacgtaggtagcaagcgttgtccggaatgactgggcgtaaagggtgcgtaggtggctgagcaagttggtagtgaaattccgaggcttaacttcggcgctactaccaagactgcccggcttgagtacaggagaggtaagtggaattcctagtgtagcggtggaatgcgtagatattaggaggaacaccggtggcgaaagcgacttactggcctgcaactgacactgaggcacgaaagcgtggggagcaaacaggattagataccctggtagtccacgccgtaaacgatgattactaggtatgggaggtatcgactccttccgtgccgcagccaacgcaataagtaatccgcctggggagtacggccgcaaggttgaaactcaaagaaattgacggggacccgcacaagcagcggagcatgtggtttaattcgacgcgacgcgaaaaaccttaccaggtcttgacatcctttgaccgcctgagagatcaggaatctttagcaatagagcagagagacaggtggtgcatggttgtcgtcagctcgtgtcgtgagatgttcggttaagtccgacaacgagcgcaacccttgtatacagttgccaatattaagttaggaactctgtataaactgccgtggctaacacggaggaaggtggggatgacgtcaaatcatcacgccccttacgacctgggccacacacgtgctacaatggctattacaaagagcagcgaaaccgcgaggtagagcgaatctcaaaaagatagtctcagttcagattgtgggctgaaacccgcccacatgaagtcggagttgctagtaatcccggatcagcatgccggggtgaatgcgttcccgggtcttgtacacaccgcccgtcacgccatgggagttcggagtacccaaagtcaacggcctaaccgcaaggggggagttgcctaaggtaatacgaatgactggggtgaagtcgtaacaaggta

SEQ ID NO: 62 - DNA, 1444 bp, Unknown
  16S rRNA(PAC001437_g)
gacgaacgctggcggcgtgcctaacacatgcaagtcgagcggggacaaggacttcggttcttgttctagcggcggacgggtgagtaacgcgtgagcaatctgtccctcacagggggataacacttggaaacaggtgctaataccgcataagaccacggtgtcgcatggctttgaggtcaaaggagcaatccggtgaggggtgagctcgtgtcccattagatagttggcggggtaacggcccaccaagtcagcgatgggtagccgacctgagagggtgatcggccacactgggactgagacacggcccagactcctacgggaggcagcagtggggaatattgggcaatgggcgaaagcctgacccagcaacgccgcgtgagggaggaaggttttcggattgtaaacctctgtccttggggaagaaggaagtgacggtacccaaggaggaagccccggctaactacgtgccagcagccgcggtaatacgtagggggcgagcgttgtccggaatgactgggcgtaaagggcgtgtaggcggccgactaagtctgatgtgaaatacccgcttttaaggtgggtcgtgcattggaaactggatggctagagtgcggaagaggtaagtggaattcccagtgtagcggtgaaatgcgtagagattgggaggaacaccagtggcgaaggcgacttactgggccgcaactgacgctgaggcgcgaaagcgtggggagcaaacaggattagataccctggtagtccacgctgtaaacgatgaatgctaggtgtagggggtatcgacccctcctgtgccgcagttaacacaataagcattccgcctggggagtacggccgcaaggttgaaactcaaagaaattgacgggggcccgcacaagcagcggagcatgtggtttaattcgaagcaacgcgaagaaccttaccaggtcttgacatccacttaaagccgtagagatacggtgtgagcttgctcaaagtgagacaggtggtgcatggttgtcgtcagctcgtgtcgtgagatgttgggttaagtcccgcaacgagcgcaacccctattatcagttactaacgtgtagaggcgaggactctgatgagactgccggggacaactcggaggaaggtggggacgacgtcaaatcatcatgccccttatgacctgggctacacacgtgctacaatggctgtaacaaagagaagcagagccgtaaggccgagcggatctcaaaaaagcagtctcagttcggattgtgggctgcaacccgcccacatgaagttggagttgctagtaatcgcggatcagcatgccgcggtgaatacgttcccgggccttgtacacaccgcccgtcacaccatgggagtttggagcacccaaagccggtgaggtaaccgcaaggagccagccgtccaaggtgagacaaatgactggggtgaa

SEQ ID NO: 63 - DNA, 1452 bp, Unknown
  16S rRNA(PAC001468_g)
gatgaacgctggcggcgtgcctaacacatgcaagtcgaacgaagatgcatttcagatcccttcggggtgacgagatgcagacttagtggcggacgggtgagtaatgtatgagcaacctgccttcaagaggggaataacagtcggaaacgactgctaataccgcataataaagcgtagtcgcatgacaatgctttcaaaggagcaatccgcttgaagatgggctcatatctgattagatagttggtgaggtaacggctcaccaagtctgcgatcagtagccggactgagaggttgaacggccacattggaactgagatacggtccagactcctacgggaggcagcagtggggaatattgggcaatgggcgaaagcctgacccagcaacgccgcgtgaaggaagaaggtcttcggattgtaaacttttgtcttatgggacgataatgacggtaccataggaggaagccacgactaactacgtgccagcagtcgcggtaatacgtaggtggcgagcgttatccggaattattgggtgtaaagggtgcgtaggcgggtcgtaaagtcagatgtgaaatgcggaggctcaacctccgaactgcatttgaaacttacgatcttgagtggagtagaggcaagcggaattcccggtgtagcggtgaaatgcatagatatcgggaggaacaccagtggcgaaggcggcttgctgggcttttactgacgctgaggcacgaaagtgtggggagcaaacaggattagataccctggtagtccacaccgtaaacgatgattactaggtgtaggtcggctgaaccggtctgtgccgcagttaacacaataagtaatccacctggggagtacggccgcaaggttgaaactcaaaggaattgacgggggcccgcacaagcagtggagtatgtggtttaattcgacgcaacgcgaaaaaccttaccaggtcttgacatccgactaacgaagtagagatacattaggtgcccttcggggaaagttgagacaggtggtgcatggttgtcgtcagctcgtgtcgtgagatgttgggttaagtcccgcaacgagcgcaacccttgttgtcagttgctacgcaagagcactctggcaagactgccgttgacaaaacggaggaaggtgaggatgacgtcaaatcatcatgccctttatgacctgggctacacacgtactacaatggcggtaaacaaagcggagcgaagtcgtgaggcagagcaaatctccaaaagccgtctcagttcagattgcaggctgaaactcgcctgcatgaagttggaattgctagtaatcgtgaatcagcatgtcacggtgaatacgttcccgggccttgtacacaccgcccgtcaaaccatgagagttgggaatgcccgaagtctgttgtctgaccgcaagggggacgcagccgaaggcaggctcgatgattggggtt

SEQ ID NO: 64 - DNA, 1439 bp, Unknown
  16S rRNA(PAC001609_g)
gatgaacgctggcggcgtgcctaacacatgcaagtcgagcgagaaatcttggaatgagacttcggttaagtgaagagatggaaagcggcggacgggtgagtaacgcgtaggcaacctgccttatgcagagggatagccattggaaacgatgattaaaacctcataatgccattttatcacatggtgagatggtcaaagatttatcggcataagatgggcctgcgtctgattagctagttggtggggtaacggcctaccaaggcgacgatcagtagccgacctgagagggtgatcggccacattggaactgagacacggtccaaactcctacgggaggcagcagtggggaatattgcacaatgggcgaaagcctgatgcagcaacgccgcgtgaaggaagaaggtcttcggatcgtaaacttctgtccttggggaagataatgacggtacccttggaggaagccccggctaactacgtgccagcagccgcggtaatacgtagggggcaagcgttatccggaattattgggcgtaaagagtgcgtaggtggttacctaagcagggggtgaaaggcactggcttaaccaatgtcagccccctgaactgggtaccttgagtgcaggagaggaaagcggaattcctagtgtagcggtgaaatgcgtagatattaggaggaacaccagtggcgaaggcggctttctggactgttactgacactgaggcacgaaagtgtggggagcaaacaggattagataccctggtagtccacaccgtaaacgatgagcactaggtgtcggggtcgcaagacttcggtgccgcagttaacgcattaagtgctccgcctggggagtacgtacgcaagtatgaaactcaaaggaattgacggggacccgcacaagcagcggagcatgtggtttaattcgaagcaacgcgaagaaccttaccaggacttgacatccctctgaaacccctgataacgaaggggcctctacggacagaggagacaggtggtgcatggttgtcgtcagctcgtgtcgtgagatgttgggttaagtcccgcaacgagcgcaacccttgctgttagttgccatcattgagttgggcactctaacgggactgccggggataactcggaggaaggtggggatgacgtcaaatcatcatgccccttatgttctgggctacacacgtgctacaatggtcggtacaaagagcagcaagaccgtgaggtggagcaaatctcaaaaaccgatcccagttcggattgcaggctgcaactcgcctgcatgaagttggagttgctagtaatcgcgaatcagaatgtcgcggtgaatgcgttcccgggtcttgtacacaccgcccgtcacaccacggaagttgggggtgcccaaagttggtcgataaatagattacctaaggacaaaaccaatgactggggtg

SEQ ID NO: 65 - DNA, 1442 bp, Unknown
  16S rRNA(PAC002148_g)
gatgaacgctggcggcgtgcttaacacattcaagtcgtacgaactgattttgaagcttgcttcggaagaaagttagtggcggacgggtgagtaacgcgtgagcaacctgcctttgtgagggggataacacagggaaacttgtgctaataccgcatgacgcatacgaaagacatctttagtatgttgaaggagcaatccgcacaaagatgggctcgcgtctgattagatagttggtggggtaacggcctaccaagtcgacgatcagtagccggactgagaggttgaacggccacattggaactgagaaacggtccagactcctacgggaggcagcagtggggaatattgggcaatgggcgaaagcctgacccagcgacgccgcgtgagggaagaaggtcttcggattgtaaacctttgtagacagggaagaagaaagtgacggtacctgtaaagtaagccacggctaactacgtgccagcagccgcggtaatacgtaggtggcaagcgttatccggatttactgggtgtaaagggtgtgtaggcggggaaacaagtcagatgtgaaatgccaaggctaaaccatggagctgcatttgaaactgtttttcttgagagtgggagaggtaagcggaattcccggtgtagcggtgaaatgcgtagatatcgggaggaacaccagtggcgaaggcggcttactggaccattactgacgctgagacacgaaagcgtggggagcaaacaggattagataccctggtagtccacgccgtaaacgatgaatactaggtgtagggggtataaacctctgtgccggagttaacacaataagtattccacctggggagtacggccgcaaggttgaaactcaaaggaattgacgggagcccgcacaagcagtggagtatgtggtttaattcgacgcaacgcgaagaaccttaccaggacttgacatcctaagaataccgagtaatgttggtagtgcccttcggggagcttagagacaggtggtgcatggttgtcgtcagctcgtgtcgtgagatgttgggttaagtcccgcaacgagcgcaacccttacgtttagttgctacgcaagagcactctgaacggactgccgttgacaaaacggaggaaggcggggacgacgtcaaatcatcatgccccttacgttctgggctacacacgtactacaatggcgtctaacagaggggagcgaaggagcgatccggagcaaatcccaaaaagacgtcccagttcagactgcaggctgcaacccgcctgcacgaagtcggaattgctagtaatcgcaggtcagcatactgcggtgaatacgttcccgggctttgtacacaccgcccgtcaaaccatgaaagtcgggaatacccgaagtcagtgagctgaccgcaagggggcagctgcctaaggtaggttcgatgattggggtt

SEQ ID NO: 66 - DNA, 1464 bp, Unknown
  16S rRNA(PAC002518_g)
gatgaacgctggcggcgtgcctaacacatgcaagtcgaacggagttatgatgtgagcgggaagtgcttgcactaaacaatcttttcataacttagtggcggacgggtgagtaacgcgtgggtaacctgccctgtactgggggacaacagttggaaacgactgctaataccgcataagcgcacgggatcgcatgatcctgtgtgaaaaactccggtggtacaggatggacccgcgtctgattagctggttggtgaggtaacggcccaccaaggcaacgatcagtagccggcctgagagggtgaacggccacattgggactgagacacggcccaaactcctacgggaggcagcagtggggaatattgcacaatgggggaaaccctgatgcagcgacgccgcgtgagtgaagaagtatttcggtatgtaaagctctatcagcagggaagaaaatgacggtacctgactaagaagccccggctaactacgtgccagcagccgcggtaatacgtagggggcaagcgttatccggatttactgggtgtaaagggagcgtagacggcatggcaagtctgaagtgaaatgcgggggctcaacccctgaactgctttggaaactgtcaggctggagtgcaggagaggtaagtggaattcctagtgtagcggtgaaatgcgtagatattaggaggaacaccagtggcgaaggcggcttactggactgtaactgacgttgaggctcgaaagcgtggggagcaaacaggattagataccctggtagtccacgccgtaaacgatgattactaggtgttggggatttataaatcctcggtgccgtcgcaaacgcaataagtaatccacctggggagtacgttcgcaagaatgaaactcaaaggaattgacggggacccgcacaagcggtggagcatgtggtttaattcgaagcaacgcgaagaaccttacctggtcttgacatcccgatgcataacgggtaatgccgttagtacttcggtacattggagacaggtggtgcatggttgtcgtcagctcgtgtcgtgagatgttgggttaagtcccgcaacgagcgcaacccttatctttagtagccagcgagcaaagtcgggcactctagagagactgccggggataacccggaggaaggtggggatgacgtcaaatcatcatgccccttatgaccagggctacacacgtgctacaatggcgtaaacaaagggaagcgaccctgtgaaggcaagcgaatcccaaaaataacgtcccagttcggattgtagtctgcaactcgactacatgaagctggaatcgctagtaatcgcgaatcagcatgtcgcggtgaatacgttcccgggtcttgtacacaccgcccgtcacaccatgggagtcggaaatgcccgaagtcggtgacctaaccgcaaggaaggagccgccgaaggcaggtctggtaactggggtg

SEQ ID NO: 67 - DNA, 1443 bp, Unknown
  16S rRNA(Paludicola genus)
gacgaacgctggcggcgcgcctaacacatgcaagtcgaacgaagtttgcaggattgatccttcgggtgattgagcgtaaacttagtggcggacgggtgagtaacacgtgagcaacctgccctacagtggggataacgttttgaaaagaacgctaataccgcataacgtatcggagaggcatctttctgataccaaaggagcaatccgctgtaagatgggctcgcgtccgattagccagttggcggggtaacggcccaccaaagcgacgatcggtagccggactgagaggttgatcggccacattgggactgagacacggcccagactcctacgggaggcagcagtgggggatattgcacaatgggggaaaccctgatgcagcgacgccgcgtgagggaagaaggtcttcggattgtaaacctctgtcttcggtgacgaaaatgacggtagccgaggaggaagccacggctaactacgtgccagcagccgcggtaatacgtaggtggcaagcgttgtccggaattactgggtgtaaagggagcgtaggcgggaatacaagttgaatgtgaaaactatgggctcaacccatagttgcgttcaaaaccgtgtttcttgagtgaagtagaggtaagcggaattcctagtgtagcggtgaaatgcgtaaatattaggaggaacaccagtggcgaaggcggcttactgggctttaactgacgctgaggctcgaaagcgtgggtagcaaacaggattagataccctggtagtccacgctgtaaacgatgattactaggtgtggggggactgaccccttccgtgccggagttaacacaataagtaatccacctggggagtacgaccgcaaggttgaaactcaaaggaattgacgggggcccgcacaagcagtggagtatgtggtttaattcgacgcaacgcgaagaaccttaccaggtcttgacatcggatgcatagctaagagattagcgaagtccttcgggacatccagacaggtggtgcatggttgtcgtcagctcgtgtcgtgagatgttgggttaagtcccgcaacgagcgcaacccttatgtttagttgctacgcaagagcactctagacagactgccgttgacaaaacggaggaaggtggggatgacgccaaatcatcatgccccttatgacctgggctacacacgtactacaatggctatcaacagagggcagcaacctcgcgagggggagcaaatctccaaaaatagtctcagttcagattgcaggctgcaactcgcctgcatgaaggcggaattgctagtaatcgcggatcagcatgccgcggtgaatacgttcccgggccttgtacacaccgcccgtcacaccatgagagttggcaacacccgaagtcagcaggctaacgcaagaagccgctgccgaaggtggggttgacgattggggtg

SEQ ID NO: 68 - DNA, 1461 bp, Unknown
  16S rRNA(Romboutsia genus)
agagtttgatcctggctcaggatgaacgctggcggcgtgcctaacacatgcaagtcgagcgatcttcttcggaagagagcggcggacgggtgagtaacgcgtgggtaacctgccctgtacacacggataacataccgaaaggtatgctaatacgagataatatgcttttatcgcatggtagaagtatcaaagctccggcggtacaggatggacccgcgtctgattagctagttggtaaggtaacggcttaccaaggcgacgatcagtagccgacctgagagggtgatcggccacattggaactgagacacggtccaaactcctacgggaggcagcagtggggaatattgcacaatgggcgaaagcctgatgcagcaacgccgcgtgagcgatgaaggccttcgggtcgtaaagctctgtcctcaaggaagataatgacggtacttgaggaggaagccccggctaactacgtgccagcagccgcggtaatacgtagggggctagcgttatccggaattactgggcgtaaagggtgcgtaggtggtttcttaagtcagaggtgaaaggctacggctcaaccgtagtaagcctttgaaactgggaaacttgagtgcaggagaggagagtggaattcctagtgtagcggtgaaatgcgtagatattaggaggaacaccagttgcgaaggcggctctctggactgtaactgacactgaggcacgaaagcgtggggagcaaacaggattagataccctggtagtccacgccgtaaacgatgagtactagctgtcggaggttacccccttcggtggcgcagctaacgcattaagtactccgcctgggaagtacgctcgcaagagtgaaactcaaaggaattgacggggacccgcacaagtagcggagcatgtggtttaattcgaagcaacgcgaagaaccttacctaagcttgacatccttttgaccgatgcctaatcgcatctttcccttcggggacagaagtgacaggtggtgcatggttgtcgtcagctcgtgtcgtgagatgttgggttaagtcccgcaacgagcgcaacccttgcctttagttgccagcattaagttgggcactctagagggactgccagggataacctggaggaaggtggggatgacgtcaaatcatcatgccccttatgcttagggctacacacgtgctacaatgggtggtacagagggcagccaagtcgtgaggcggagctaatcccttaaagccattctcagttcggattgtaggctgaaactcgcctacatgaagctggagttactagtaatcgcagatcagaatgctgcggtgaatgcgttcccgggtcttgtacacaccgcccgtcacaccacgggagttgggggcgcccgaagccggattgctaaccttttggaagcgtccgtcgaaggtgaaatcaataactggggtgaagtcgtaacaaggta

SEQ ID NO: 69 - DNA, 1361 bp, Unknown
  16S rRNA(Roseburia genus)
agagtttgatcctggctcaggatgaacgctggcggcgtgcttaacacatgcaagtcgaacgaagcactctatttgattttcttcggaaatgaagattttgtgactgagtggcggacgggtgagtaacgcgtgggtaacctgcctcatacagggggataacagttggaaacgactgctaataccgcataagcgcacagtactgcatggtaccgtgtgaaaaactccggtggtatgagatggacccgcgtctgattagccagttggcggggtaacggcccaccaaagcgacgatcagtagccgacctgagagggtgaccggccacattgggactgagacacggccnnaactcctrcgggaggcagcagtggggaatattgcnnaatgggggaaaccctnatgcagcgacgccgcgtgagcgaagaagtatttcggtatgtaaagctctatcagcagggaagaaaaatgacggtacctgactaagaagcaccggctaaatacgtgccagcagccgcggtaatacgtatggtgcmagcgttatycggatttactgggtgtmaagggagcgcmggcggtgcggcaagtctgatgtgaaagnccggggctymaccccggnactgcattggaaactgtcgtactagagtgtyggaggggnaagtggnattcctagtgtagcggtgaaatgcgtagatattaggaggaacaccagtggcgaaggcggcttactggacgattactgacgctgaggctcgaaagcgtggggagcaaacaggattagataccctggtagtccacgccgtaaacgatgaatactaggtgtcggggagcattgctcttcggtgccgcagcaaacgcwataagtattccncctggggagtacgttcgcaagaatgaaactcaaaggaattgacggggacccgcncnagcggtggagcatgtggtttaattcgaagnaacgcgaagaaccttaccaagtcttgacatccttctgacaatrtatgtaatgtatattctcttcggagcagaagtgacaggtggtgcatggttgtcgtcagctngtgtcgtgagatgttgggttaagtcccgcaacgagcgcaaccctyattcttagtagccagcggttcggccgggcactctagggagactgccagggataacctggaggaaggtggggatgacgtcaaatcatcatgccccttatgacttgggctacacacgtgctacaatggcgtaaacnaagggaagcaagaccgtgaggtggagcaaaccccaaaaataacgtctcagttcggactgtagtctgcaactcgactacacgaagctggaatcgctagtaatcgcgaatcmgaatgncgcggtgaat

SEQ ID NO: 70 - DNA, 1471 bp, Unknown
  16S rRNA(Ruminococcaceae_uc)
agagtttgatcctggctcaggacgaacgctggcggcacgcttaacacatgcaagtcgaacggagataatttgagtttacttaggttatcttagtggcggacgggtgagtaacacgtgagcaacctaccttagagagagggatagcttctggaaacggatggtaatacctcataacataactgaaccgcatgatttagttatcaaagatttatcactctgagatgggctcgcgtctgattagatagttggtgaggtaacggctcaccaagtcgacgatcagtagccggactgagaggttgaacggccacattgggactgagacacggcccagactcctacgggaggcagcagtggggaatattgcacaatgggggaaaccctgatgcagcgatgccgcgtggaggaagaaggttttcggattgtaaactcctgtcttaaaggacgataatgacggtactttaggaggaagctccggctaactacgtgccagcagccgcggtaatacgtagggagcgagcgttgtccggaattactgggtgtaaagggagcgtaggcgggagcgcaagtcagatgtgaaatacatgggctcaacccatgggctgcatttgaaactgtgtttcttgagtgaagtagaggtaagcggaattcctggtgtagcggtgaaatgcgtagatatcaggaggaacaccggtggcgaaggcggcttactgggcttttactgacgctgaggctcgaaagcgtggggagcaaacaggattagataccctggtagtccacgctgtaaacgatgattactaggtgtggggggactgaccccttccgtgccgcagttaacacaataagtaatccacctggggagtacggccgcaaggttgaaactcaaaggaattgacgggggcccgcacaagcagtggagtatgtggtttaattcgaagcaacgcgaagaaccttaccaggtcttgacatcgtatgcatagtctagagatagatgaaattccttcggggacatatagacaggtggtgcatggttgtcgtcagctcgtgtcgtgagatgttgggttaagtcccgcaacgagcgcaacccttacctttagttgctacgcaagagcactctaaagggactgccgttgacaaaacggaggaaggtggggatgacgtcaaatcatcatgccccttatgacctgggctacacacgtactacaatggcaattaacaaagagaagcaagacggtgacgtggagcgaatctcaaaaaattgtcccagttcagattgcaggctgcaactcgcctgcatgaagtcggaattgctagtaatcgcggatcagcatgccgcggtgaatacgttcccgggccttgtacacaccgcccgtcacaccatgggagtcggtaacacccgaagtcggtagtctaacagcaatgaggacgccgccgaaggtgggattgatgactggggtgaagtcgtaacaaggta

SEQ ID NO: 71 - DNA, 1470 bp, Unknown
  16S rRNA(Ruminococcus genus)
agagtttgatcctggctcaggacgaacgctggcggcacgcttaacacatgcaagtcgaacgagagaagaggagcttgcttttctgatctagtggcggacgggtgagtaacacgtgagcaatctgcctttcagagggggataccgattggaaacgatcgttaataccgcataacataattgaaccgcatgatttgattatcaaagatttatcgctgaaagatgagctcgcgtctgattagctagttggtaaggtaacggcttaccaaggcgacgatcagtagccggactgagaggttgatcggccacattgggactgagacacggcccagactcctacgggaggcagcagtggggaatattgcacaatggaggaaactctgatgcagcgatgccgcgtgagggaagaaggttttaggattgtaaacctctgtcttcagggacgaaaaaagacggtacctgaggaggaagctccggctaactacgtgccagcagccgcggtaatacgtagggagcgagcgttgtccggaattactgggtgtaaagggagcgtaggcgggatcgcaagtcagatgtgaaaactatgggcttaacccataaactgcatttgaaactgtggttcttgagtgaagtagaggtaagcggaattcctagtgtagcggtgaaatgcgtagatattaggaggaacatcagtggcgaaggcggcttactgggctttaactgacgctgaggctcgaaagcgtggggagcaaacaggattagataccctggtagtccacgccgtaaacgatgattactaggtgtggggggactgaccccttccgtgccgcagcaaacgcaataagtaatccacctggggagtacgaccgcaaggttgaaactcaaaggaattgacgggggcccgcacaagcagtggagtatgtggattaattcgaagcaacgcgaagaaccttaccaggtcttgacatcgtatgcatagctcagagatgagtgaaatctcttcggagacatatagacaggtggtgcatggttgtcgtcagctcgtgtcgtgagatgttgggttaagtcccgcaacgagcgcaacccttactgttagttgctacgcaagagcactctagcaggactgccgttgacaaaacggaggaaggtggggatgacgtcaaatcatcatgccccttatgacctgggcctcacacgtactacaatggctgtcaacagagggaagcaaagccgcgaggtggagcgaacccctaaaagcagtcttagttcggattgtaggctgcaacccgcctacatgaagtcggaattgctagtaatcgcagatcagcatgctgcggtgaatacgttcccgggccttgtacacaccgcccgtcacgccatgggagtcggtaacacccgaagcctgtagtctaaccgcaaggaggacgcagtcgaaggtgggattgatgactggggtgaagtcgtaacaaggta

SEQ ID NO: 72 - DNA, 1458 bp, Unknown
  16S rRNA(Ruminococcus_g2)
ggcggcgtgcctaacacatgcaagtcgaacggaactgttttgaaagatttcttcggaatgaatttgatttagtttagtggcggacgggtgagtaacgcgtgagtaacctgccttcaagagggggataacattctgaaaagaatgctaataccgcatgacatatcggaaccacatggttctgatatcaaagattttatcgcttgaagatggactcgcgtccgattagttagttggtgaggtaacggctcaccaagaccgcgatcggtagccggactgagaggttgaacggccacattgggactgagacacggcccagactcctacgggaggcagcagtgggggatattgcgcaatgggggcaaccctgacgcagcaacgccgcgtgaaggatgaaggttttcggattgtaaacttcttttattaaggacgaaaaatgacggtacttaatgaataagctccggctaactacgtgccagcagccgcggtaatacgtagggagcaagcgttgtccggatttactgggtgtaaagggtgcgtaggcggctttgcaagtcagatgtgaaatctatgggctcaacccataaactgcatttgaaactgtagagcttgagtgaagtagaggcaggcggaattccccgtgtagcggtgaaatgcgtagagatggggaggaacaccagtggcgaaggcggcctgctgggctttaactgacgctgaggcacgaaagcgtgggtagcaaacaggattagataccctggtagtccacgctgtaaacgatgattactaggtgtggggggtctgaccccttccgtgccggagttaacacaataagtaatccacctggggagtacggccgcaaggttgaaactcaaaggaattgacgggggcccgcacaagcagtggagtatgtggtttaattcgaagcaacgcgaagaaccttaccaggtcttgacatccaactaacgaagtagagatacattaggtgcccttcggggaaagttgagacaggtggtgcatggttgtcgtcagctcgtgtcgtgagatgttgggttaagtcccgcaacgagcgcaacccttgctattagttgctacgcaagagcactctaataggactgccgttgacaaaacggaggaaggtggggacgacgtcaaatcatcatgccccttatgacctgggctacacacgtactacaatggctgttaacagagggaagcaagacagtgatgtggagcaaacccctaaaaacattctcagttcagattgcaggctgcaacccgcctgcatgaagatggaattgctagtaatcgcggatcagaatgccgcggtgaatacgttcccgggccttgtacacaccgcccgtcacaccatgggagccggtaatacccgaagtcagtagtccaacctcgtgaggacgctgccgaaggtaggattggcgactggggtgaagtcgtaacaaggta

SEQ ID NO: 73 - DNA, 1453 bp, Unknown
  16S rRNA(Sporobacter genus)
gatgaacgctggcggcgtgcctaacacatgcaagtcgaacggagttactttggtgaagttttcggatggatctgatttaacttagtggcggacgggtgagtaatgcgtgagcaacctgcccttcagagggggacaacagttggaaacgactgctaataccgcataatgtatccgggaggcatctcctggataccaaaggagaaatccgctgatggatgggctcacgtctgattagctagttggtgaggtaacggctcaccaaggctgcgatcagtagccggactgagaggttgaacggccacattgggactgagatacggcccagactcctacgggaggcagcagtggggaatattgggcaatgggcgaaagcctgacccagcaacgccgcgtgaaggaagaaggccttcgggttgtaaacttcttttaagagggacgaagaagtgacggtacctcttgaataagccacggctaactacgtgccagcagccgcggtaatacgtaggtggcgagcgttatccggatttactgggtgtaaagggcgcgtaggcgggaatgcaagtcagatgtgaaatccaagggctcaacccttgaactgcatttgaaactgtatttcttgagtgtcggagaggttgacggaattcctagtgtagcggtgaaatgcgtagatattaggaggaacaccagtggcgaaggcggtcaactggacgataactgacgctgaggcgcgaaagcgtggggagcaaacaggattagataccctggtagtccacgccgtaaacgatgaatactaggtgtggggggactgaccccttccgtgccgcagttaacacaataagtattccacctggggagtacgaccgcaaggttgaaactcaaaggaattgacgggggcccgcacaagcagtggattatgtggtttaattcgaagcaacgcgaagaaccttaccagggcttgacatccaactaacgaagcagagatgcattaggtgcccttcggggaaagttgagacaggtggtgcatggttgtcgtcagctcgtgtcgtgagatgttgggttaagtcccgcaacgagcgcaacccctattgttagttgctacgcaagagcactctagcgagactgccgttgacaaaacggaggaaggtggggacgacgtcaaatcatcatgccccttatgtcctgggctacacacgtaatacaatggcatttaacagagggaagcaaaaccgcgaggtagagcaaatccctaaaaggtgtctcagttcggattgcaggctgcaactcgcctgcatgaagtcggaattgctagtaatcgcggatcagcatgccgcggtgaatacgttcccgggccttgtacacaccgcccgtcacaccatgagagtcgggaacacccgaagtccgtagcttaaccgcaaggagggcgcggccgaaggtgggttcgataattggggtg

SEQ ID NO: 74 - DNA, 1487 bp, Unknown
  16S rRNA(Subdoligranulum genus)
agagtttgatcctggctcaggacgaacgctggcggcgcgcctaacacatgcaagtcgaacggagttatttcggttgaagttttcggatggatactggtttaacttagtggcgaacgggtgagtaacgcgtgagtaacctgccctggagtgggggacaacagttggaaacgactgctaataccgcataagcccacggcccggcatcgggctgagggaaaaggatttattcgcttcaggatggactcgcgtccaattagctagttggtgaggtaacggcccaccaaggcgacgattggtagccggactgagaggttgaacggccacattgggactgagacacggcccagactcctacgggaggcagcagtgggggatattgcacaatgggggaaaccctgatgcagcgacgccgcgtggaggaagaaggttttcggattgtaaactcctgtcgttagggacgaatcttgacggtacctaacaagaaagcaccggctaactacgtgccagcagccgcggtaaaacgtagggtgcaagcgttgtccggaattactgggtgtaaagggagcgcaggcggaccggcaagttggaagtgaaatctatgggctcaacccataaattgctttcaaaactgctggccttgagtagtgcagaggtaggtggaattcccggtgtagcggtggaatgcgtagatatcgggaggaacaccagtggcgaaggcgacctactgggcaccaactgacgctgaggctcgaaagcatgggtagcaaacaggattagataccctggtagtccatgccgtaaacgatgattactaggtgttggaggattgaccccttcagtgccgcagttaacacaataagtaatccacctggggagtacgaccgcaaggttgaaactcaaaggaattgacgggggcccgcacaagcagtggagtatgtggtttaattcgaagcaacgcgaagaaccttaccaggtcttgacatccgatgcatagtgcagagatgcatgaagtccttcgggacatcgagacaggtggtgcatggttgtcgtcagctcgtgtcgtgagatgttgggttaagtcccgcaacgagcgcaacccttattgccagttactacgcaagaggactctggcgagactgccgttgacaaaacggaggaaggtggggatgacgtcaaatcatcatgccctttatgacctgggctacacacgtactacaatggcgtttaacaaagagaagcaagaccgcgaggtggagcaaaactcaaaaacaacgtctcagttcagattgcaggctgcaactcgcctgcatgaagtcggaattgctagtaatcgcggatcagcatgccgcggtgaatacgttcccgggccttgtacacaccgcccgtcacaccatgagagccggggggacccgaagtcggtagtctaaccgcaaggaggacgccgccgaaggtaaaactggtgattggggtgaagtcgtaacaaggta

SEQ ID NO: 75 - DNA, 17 bp, Artificial Sequence
  forward universal primer
cctacgggnggcwgcag

SEQ ID NO: 76 - DNA, 21 bp, Artificial Sequence
  reverse universal primer
gactachvgggtatctaatcc